European Patent Application EP 4 714 980 A1, published March 25, 2026. Title: 用于治疗补体旁路相关疾病的AAV载体. Applicant: 合肥星眸生物科技有限公司. The sequence listing filed with the application follows.

SEQUENCE LISTING (82 sequences)

SEQ ID NO: 1 - protein, 249 aa, synthetic construct
CGSPPPILNGRISYYSTPIAVGTVIRYSCSGTFRLIGEKSLLCITKDKVDGTWDKPAPKCEYFNKYSSCPEPIVPGGYKIRGSTPYRHGDSVTFACKTNFSMNGNKSVWCQANNMWGPTRLPTCVSVFPLECPALPMIHNGHHTSENVGSIAPGLSVTYSCESGYLLVGEKIINCLSSGKWSAVPPTCEEARCKSLGRFPNGKVKEPPILRVGVTANFFCDEGYRLQGPPSSRCVIAGQGVAWTKMPVC

SEQ ID NO: 2 - protein, 242 aa, synthetic construct
CNELPPRRNTEILTGSWSDQTYPEGTQAIYKCRPGYRSLGNVIMVCRKGEWVALNPLRKCQKRPCGHPGDTPFGTFTLTGGNVFEYGVKAVYTCNEGYQLLGEINYRECDTDGWTNDIPICEVVKCLPVTAPENGKIVSSAMEPDREYHFGQAVRFVCNSGYKIEGDEEMHCSDDGFWSKEKPKCVEISCKSPDVINGSPISQKIIYKENERFQYKCNMGYEYSERGDAVCTESGWRPLPSC

SEQ ID NO: 3 - protein, 58 aa, synthetic construct
CSKSSIDIENGFISESQYTYALKEKAKYQCKLGYVTADGETSGSITCGKDGWSAQPTC

SEQ ID NO: 4 - protein, 120 aa, synthetic construct
CGPPPPIDNGDITSFPLSVYAPASSVEYQCQNLYQLEGNKRITCRNGQWSEPPKCLHPCVISREIMENYNIALRWTAKQKLYSRTGESVEFVCKRGYRLSSRSHTLRTTCWDGKLEYPTC

SEQ ID NO: 5 - protein, 695 aa, synthetic construct
CGSPPPILNGRISYYSTPIAVGTVIRYSCSGTFRLIGEKSLLCITKDKVDGTWDKPAPKCEYFNKYSSCPEPIVPGGYKIRGSTPYRHGDSVTFACKTNFSMNGNKSVWCQANNMWGPTRLPTCVSVFPLECPALPMIHNGHHTSENVGSIAPGLSVTYSCESGYLLVGEKIINCLSSGKWSAVPPTCEEARCKSLGRFPNGKVKEPPILRVGVTANFFCDEGYRLQGPPSSRCVIAGQGVAWTKMPVCGGGGSGGGGSEDCNELPPRRNTEILTGSWSDQTYPEGTQAIYKCRPGYRSLGNVIMVCRKGEWVALNPLRKCQKRPCGHPGDTPFGTFTLTGGNVFEYGVKAVYTCNEGYQLLGEINYRECDTDGWTNDIPICEVVKCLPVTAPENGKIVSSAMEPDREYHFGQAVRFVCNSGYKIEGDEEMHCSDDGFWSKEKPKCVEISCKSPDVINGSPISQKIIYKENERFQYKCNMGYEYSERGDAVCTESGWRPLPSCEIRVKTCSKSSIDIENGFISESQYTYALKEKAKYQCKLGYVTADGETSGSITCGKDGWSAQPTCIKSDSTGKCGPPPPIDNGDITSFPLSVYAPASSVEYQCQNLYQLEGNKRITCRNGQWSEPPKCLHPCVISREIMENYNIALRWTAKQKLYSRTGESVEFVCKRGYRLSSRSHTLRTTCWDGKLEYPTC

SEQ ID NO: 6 - protein, 724 aa, synthetic construct
MPMGSLQPLATLYLLGMLVASCLGISCGSPPPILNGRISYYSTPIAVGTVIRYSCSGTFRLIGEKSLLCITKDKVDGTWDKPAPKCEYFNKYSSCPEPIVPGGYKIRGSTPYRHGDSVTFACKTNFSMNGNKSVWCQANNMWGPTRLPTCVSVFPLECPALPMIHNGHHTSENVGSIAPGLSVTYSCESGYLLVGEKIINCLSSGKWSAVPPTCEEARCKSLGRFPNGKVKEPPILRVGVTANFFCDEGYRLQGPPSSRCVIAGQGVAWTKMPVCGGGGSGGGGSEDCNELPPRRNTEILTGSWSDQTYPEGTQAIYKCRPGYRSLGNVIMVCRKGEWVALNPLRKCQKRPCGHPGDTPFGTFTLTGGNVFEYGVKAVYTCNEGYQLLGEINYRECDTDGWTNDIPICEVVKCLPVTAPENGKIVSSAMEPDREYHFGQAVRFVCNSGYKIEGDEEMHCSDDGFWSKEKPKCVEISCKSPDVINGSPISQKIIYKENERFQYKCNMGYEYSERGDAVCTESGWRPLPSCEIRVKTCSKSSIDIENGFISESQYTYALKEKAKYQCKLGYVTADGETSGSITCGKDGWSAQPTCIKSDSTGKCGPPPPIDNGDITSFPLSVYAPASSVEYQCQNLYQLEGNKRITCRNGQWSEPPKCLHPCVISREIMENYNIALRWTAKQKLYSRTGESVEFVCKRGYRLSSRSHTLRTTCWDGKLEYPTCAKR

SEQ ID NO: 7 - protein, 181 aa, synthetic construct
CVNPPTVQNAYIVSRQMSKYPSGERVRYQCRSPYEMFGDEEVMCLNGNWTEPPQCKDSTGKCGPPPPIDNGDITSFPLSVYAPASSVEYQCQNLYQLEGNKRITCRNGQWSEPPKCLHPCVISREIMENYNIALRWTAKQKLYSRTGESVEFVCKRGYRLSSRSHTLRTTCWDGKLEYPTC

SEQ ID NO: 8 - protein, 689 aa, synthetic construct
CGSPPPILNGRISYYSTPIAVGTVIRYSCSGTFRLIGEKSLLCITKDKVDGTWDKPAPKCEYFNKYSSCPEPIVPGGYKIRGSTPYRHGDSVTFACKTNFSMNGNKSVWCQANNMWGPTRLPTCVSVFPLECPALPMIHNGHHTSENVGSIAPGLSVTYSCESGYLLVGEKIINCLSSGKWSAVPPTCEEARCKSLGRFPNGKVKEPPILRVGVTANFFCDEGYRLQGPPSSRCVIAGQGVAWTKMPVCGGGGSGGGGSEDCNELPPRRNTEILTGSWSDQTYPEGTQAIYKCRPGYRSLGNVIMVCRKGEWVALNPLRKCQKRPCGHPGDTPFGTFTLTGGNVFEYGVKAVYTCNEGYQLLGEINYRECDTDGWTNDIPICEVVKCLPVTAPENGKIVSSAMEPDREYHFGQAVRFVCNSGYKIEGDEEMHCSDDGFWSKEKPKCVEISCKSPDVINGSPISQKIIYKENERFQYKCNMGYEYSERGDAVCTESGWRPLPSCERDTSCVNPPTVQNAYIVSRQMSKYPSGERVRYQCRSPYEMFGDEEVMCLNGNWTEPPQCKDSTGKCGPPPPIDNGDITSFPLSVYAPASSVEYQCQNLYQLEGNKRITCRNGQWSEPPKCLHPCVISREIMENYNIALRWTAKQKLYSRTGESVEFVCKRGYRLSSRSHTLRTTCWDGKLEYPTC

SEQ ID NO: 9 - protein, 718 aa, synthetic construct
MPMGSLQPLATLYLLGMLVASCLGISCGSPPPILNGRISYYSTPIAVGTVIRYSCSGTFRLIGEKSLLCITKDKVDGTWDKPAPKCEYFNKYSSCPEPIVPGGYKIRGSTPYRHGDSVTFACKTNFSMNGNKSVWCQANNMWGPTRLPTCVSVFPLECPALPMIHNGHHTSENVGSIAPGLSVTYSCESGYLLVGEKIINCLSSGKWSAVPPTCEEARCKSLGRFPNGKVKEPPILRVGVTANFFCDEGYRLQGPPSSRCVIAGQGVAWTKMPVCGGGGSGGGGSEDCNELPPRRNTEILTGSWSDQTYPEGTQAIYKCRPGYRSLGNVIMVCRKGEWVALNPLRKCQKRPCGHPGDTPFGTFTLTGGNVFEYGVKAVYTCNEGYQLLGEINYRECDTDGWTNDIPICEVVKCLPVTAPENGKIVSSAMEPDREYHFGQAVRFVCNSGYKIEGDEEMHCSDDGFWSKEKPKCVEISCKSPDVINGSPISQKIIYKENERFQYKCNMGYEYSERGDAVCTESGWRPLPSCERDTSCVNPPTVQNAYIVSRQMSKYPSGERVRYQCRSPYEMFGDEEVMCLNGNWTEPPQCKDSTGKCGPPPPIDNGDITSFPLSVYAPASSVEYQCQNLYQLEGNKRITCRNGQWSEPPKCLHPCVISREIMENYNIALRWTAKQKLYSRTGESVEFVCKRGYRLSSRSHTLRTTCWDGKLEYPTCAKR

SEQ ID NO: 10 - protein, 758 aa, synthetic construct
CGSPPPILNGRISYYSTPIAVGTVIRYSCSGTFRLIGEKSLLCITKDKVDGTWDKPAPKCEYFNKYSSCPEPIVPGGYKIRGSTPYRHGDSVTFACKTNFSMNGNKSVWCQANNMWGPTRLPTCVSVFPLECPALPMIHNGHHTSENVGSIAPGLSVTYSCESGYLLVGEKIINCLSSGKWSAVPPTCEEARCKSLGRFPNGKVKEPPILRVGVTANFFCDEGYRLQGPPSSRCVIAGQGVAWTKMPVCGGGGSGGGGSEDCNELPPRRNTEILTGSWSDQTYPEGTQAIYKCRPGYRSLGNVIMVCRKGEWVALNPLRKCQKRPCGHPGDTPFGTFTLTGGNVFEYGVKAVYTCNEGYQLLGEINYRECDTDGWTNDIPICEVVKCLPVTAPENGKIVSSAMEPDREYHFGQAVRFVCNSGYKIEGDEEMHCSDDGFWSKEKPKCVEISCKSPDVINGSPISQKIIYKENERFQYKCNMGYEYSERGDAVCTESGWRPLPSCEGGGGSGGGGSEDCNELPPRRNTEILTGSWSDQTYPEGTQAIYKCRPGYRSLGNVIMVCRKGEWVALNPLRKCQKRPCGHPGDTPFGTFTLTGGNVFEYGVKAVYTCNEGYQLLGEINYRECDTDGWTNDIPICEVVKCLPVTAPENGKIVSSAMEPDREYHFGQAVRFVCNSGYKIEGDEEMHCSDDGFWSKEKPKCVEISCKSPDVINGSPISQKIIYKENERFQYKCNMGYEYSERGDAVCTESGWRPLPSC

SEQ ID NO: 11 - protein, 785 aa, synthetic construct
MPMGSLQPLATLYLLGMLVASCLGISCGSPPPILNGRISYYSTPIAVGTVIRYSCSGTFRLIGEKSLLCITKDKVDGTWDKPAPKCEYFNKYSSCPEPIVPGGYKIRGSTPYRHGDSVTFACKTNFSMNGNKSVWCQANNMWGPTRLPTCVSVFPLECPALPMIHNGHHTSENVGSIAPGLSVTYSCESGYLLVGEKIINCLSSGKWSAVPPTCEEARCKSLGRFPNGKVKEPPILRVGVTANFFCDEGYRLQGPPSSRCVIAGQGVAWTKMPVCGGGGSGGGGSEDCNELPPRRNTEILTGSWSDQTYPEGTQAIYKCRPGYRSLGNVIMVCRKGEWVALNPLRKCQKRPCGHPGDTPFGTFTLTGGNVFEYGVKAVYTCNEGYQLLGEINYRECDTDGWTNDIPICEVVKCLPVTAPENGKIVSSAMEPDREYHFGQAVRFVCNSGYKIEGDEEMHCSDDGFWSKEKPKCVEISCKSPDVINGSPISQKIIYKENERFQYKCNMGYEYSERGDAVCTESGWRPLPSCEGGGGSGGGGSEDCNELPPRRNTEILTGSWSDQTYPEGTQAIYKCRPGYRSLGNVIMVCRKGEWVALNPLRKCQKRPCGHPGDTPFGTFTLTGGNVFEYGVKAVYTCNEGYQLLGEINYRECDTDGWTNDIPICEVVKCLPVTAPENGKIVSSAMEPDREYHFGQAVRFVCNSGYKIEGDEEMHCSDDGFWSKEKPKCVEISCKSPDVINGSPISQKIIYKENERFQYKCNMGYEYSERGDAVCTESGWRPLPSCE

SEQ ID NO: 12 - protein, 503 aa, synthetic construct
CGSPPPILNGRISYYSTPIAVGTVIRYSCSGTFRLIGEKSLLCITKDKVDGTWDKPAPKCEYFNKYSSCPEPIVPGGYKIRGSTPYRHGDSVTFACKTNFSMNGNKSVWCQANNMWGPTRLPTCVSVFPLECPALPMIHNGHHTSENVGSIAPGLSVTYSCESGYLLVGEKIINCLSSGKWSAVPPTCEEARCKSLGRFPNGKVKEPPILRVGVTANFFCDEGYRLQGPPSSRCVIAGQGVAWTKMPVCGGGGSGGGGSEDCNELPPRRNTEILTGSWSDQTYPEGTQAIYKCRPGYRSLGNVIMVCRKGEWVALNPLRKCQKRPCGHPGDTPFGTFTLTGGNVFEYGVKAVYTCNEGYQLLGEINYRECDTDGWTNDIPICEVVKCLPVTAPENGKIVSSAMEPDREYHFGQAVRFVCNSGYKIEGDEEMHCSDDGFWSKEKPKCVEISCKSPDVINGSPISQKIIYKENERFQYKCNMGYEYSERGDAVCTESGWRPLPSC

SEQ ID NO: 13 - protein, 530 aa, synthetic construct
MPMGSLQPLATLYLLGMLVASCLGISCGSPPPILNGRISYYSTPIAVGTVIRYSCSGTFRLIGEKSLLCITKDKVDGTWDKPAPKCEYFNKYSSCPEPIVPGGYKIRGSTPYRHGDSVTFACKTNFSMNGNKSVWCQANNMWGPTRLPTCVSVFPLECPALPMIHNGHHTSENVGSIAPGLSVTYSCESGYLLVGEKIINCLSSGKWSAVPPTCEEARCKSLGRFPNGKVKEPPILRVGVTANFFCDEGYRLQGPPSSRCVIAGQGVAWTKMPVCGGGGSGGGGSEDCNELPPRRNTEILTGSWSDQTYPEGTQAIYKCRPGYRSLGNVIMVCRKGEWVALNPLRKCQKRPCGHPGDTPFGTFTLTGGNVFEYGVKAVYTCNEGYQLLGEINYRECDTDGWTNDIPICEVVKCLPVTAPENGKIVSSAMEPDREYHFGQAVRFVCNSGYKIEGDEEMHCSDDGFWSKEKPKCVEISCKSPDVINGSPISQKIIYKENERFQYKCNMGYEYSERGDAVCTESGWRPLPSCE

SEQ ID NO: 14 - protein, 300 aa, synthetic construct
CNELPPRRNTEILTGSWSDQTYPEGTQAIYKCRPGYRSLGNVIMVCRKGEWVALNPLRKCQKRPCGHPGDTPFGTFTLTGGNVFEYGVKAVYTCNEGYQLLGEINYRECDTDGWTNDIPICEVVKCLPVTAPENGKIVSSAMEPDREYHFGQAVRFVCNSGYKIEGDEEMHCSDDGFWSKEKPKCVEISCKSPDVINGSPISQKIIYKENERFQYKCNMGYEYSERGDAVCTESGWRPLPSCEEKSCDNPYIPNGDYSPLRIKHRTGDEITYQCRNGFYPATRGNTAKCTSTGWIPAPRC

SEQ ID NO: 15 - protein, 561 aa, synthetic construct
CGSPPPILNGRISYYSTPIAVGTVIRYSCSGTFRLIGEKSLLCITKDKVDGTWDKPAPKCEYFNKYSSCPEPIVPGGYKIRGSTPYRHGDSVTFACKTNFSMNGNKSVWCQANNMWGPTRLPTCVSVFPLECPALPMIHNGHHTSENVGSIAPGLSVTYSCESGYLLVGEKIINCLSSGKWSAVPPTCEEARCKSLGRFPNGKVKEPPILRVGVTANFFCDEGYRLQGPPSSRCVIAGQGVAWTKMPVCGGGGSGGGGSEDCNELPPRRNTEILTGSWSDQTYPEGTQAIYKCRPGYRSLGNVIMVCRKGEWVALNPLRKCQKRPCGHPGDTPFGTFTLTGGNVFEYGVKAVYTCNEGYQLLGEINYRECDTDGWTNDIPICEVVKCLPVTAPENGKIVSSAMEPDREYHFGQAVRFVCNSGYKIEGDEEMHCSDDGFWSKEKPKCVEISCKSPDVINGSPISQKIIYKENERFQYKCNMGYEYSERGDAVCTESGWRPLPSCEEKSCDNPYIPNGDYSPLRIKHRTGDEITYQCRNGFYPATRGNTAKCTSTGWIPAPRC

SEQ ID NO: 16 - protein, 590 aa, synthetic construct
MPMGSLQPLATLYLLGMLVASCLGISCGSPPPILNGRISYYSTPIAVGTVIRYSCSGTFRLIGEKSLLCITKDKVDGTWDKPAPKCEYFNKYSSCPEPIVPGGYKIRGSTPYRHGDSVTFACKTNFSMNGNKSVWCQANNMWGPTRLPTCVSVFPLECPALPMIHNGHHTSENVGSIAPGLSVTYSCESGYLLVGEKIINCLSSGKWSAVPPTCEEARCKSLGRFPNGKVKEPPILRVGVTANFFCDEGYRLQGPPSSRCVIAGQGVAWTKMPVCGGGGSGGGGSEDCNELPPRRNTEILTGSWSDQTYPEGTQAIYKCRPGYRSLGNVIMVCRKGEWVALNPLRKCQKRPCGHPGDTPFGTFTLTGGNVFEYGVKAVYTCNEGYQLLGEINYRECDTDGWTNDIPICEVVKCLPVTAPENGKIVSSAMEPDREYHFGQAVRFVCNSGYKIEGDEEMHCSDDGFWSKEKPKCVEISCKSPDVINGSPISQKIIYKENERFQYKCNMGYEYSERGDAVCTESGWRPLPSCEEKSCDNPYIPNGDYSPLRIKHRTGDEITYQCRNGFYPATRGNTAKCTSTGWIPAPRCTLK

SEQ ID NO: 17 - protein, 24 aa, synthetic construct
MPMGSLQPLATLYLLGMLVASCLG

SEQ ID NO: 18 - DNA, 747 bp, synthetic construct
  source 1..747: mol_type = other DNA
tgcggctctcctccacccattctcaatggaaggatctcctactacagcacccccatagctgtcggcaccgttatccgatacagttgttccggtactttccggcttatcggcgaaaagtctttgctgtgcattaccaaggataaagtggacgggacttgggacaaacccgcacctaagtgcgagtattttaacaaatatagcagctgccctgagcctatagtacccggggggtataaaatccggggctctactccctatcgtcatggcgattctgtgaccttcgcatgtaaaactaatttttcaatgaatggcaacaagtctgtatggtgtcaagcaaataacatgtggggacctacccgcctgccaacctgtgtgtcagtgtttcccctggaatgtccagccctccctatgatccacaacggacatcacaccagcgaaaacgttggctccatcgcaccagggctctctgtgacttactcttgcgagtccgggtacctgctcgtgggtgaaaagatcatcaactgcctcagtagtggtaaatggtccgccgtgcctcccacatgtgaagaggcccggtgcaagagcctgggccggttccccaacggaaaagtgaaggaacctcctatcttgagggttggtgtgaccgctaactttttctgcgacgaggggtacaggctccaagggcctccctctagtcggtgcgtaatcgccggtcaaggagtcgcatggactaagatgcctgtgtgt

SEQ ID NO: 19 - DNA, 726 bp, synthetic construct
  source 1..726: mol_type = other DNA
tgcaacgaactgcctcctagaagaaacaccgaaatcctcacaggctcctggtcagatcagacctaccctgagggtacacaggccatctataaatgccgcccgggttaccgctccttgggcaatgttattatggtctgccggaaaggggaatgggtggccttgaaccccctcagaaagtgccaaaaaagaccctgcggacatccaggagacacacctttcgggacatttaccttgaccggtggtaacgtgttcgagtacggagtgaaggcagtctatacttgcaatgagggctaccagctcctgggggaaataaattatcgcgaatgtgatacagacggctggacgaacgacattcctatctgtgaggtggtcaaatgtctgcccgtcactgctcctgaaaacggcaagatagtgagttctgcaatggagccggatagggagtatcattttggtcaggccgtgcgctttgtgtgcaatagtgggtataaaatcgagggggatgaagaaatgcactgtagcgacgatggattctggtctaaagagaaacctaagtgtgtggagattagttgcaagagtccagacgtgattaacggtagccccatttcccaaaagataatatacaaggaaaacgaaagattccagtataaatgcaacatgggctacgagtatagcgagcggggcgatgccgtgtgtactgaaagcggctggcgccccctgccttcctgc

SEQ ID NO: 20 - DNA, 174 bp, synthetic construct
  source 1..174: mol_type = other DNA
tgttccaaaagcagcatcgacatcgaaaacggctttatatccgagagccagtatacgtatgcgctgaaggaaaaggccaagtatcagtgcaagctcggttatgtcacagctgatggcgagacctccgggtctatcacatgcggcaaagacggctggtccgctcagcctacctgc

SEQ ID NO: 21 - DNA, 360 bp, synthetic construct
  source 1..360: mol_type = other DNA
tgtgggccacctcccccaattgataatggtgatataacctccttccctcttagtgtttacgccccagcatccagcgtggagtatcaatgccaaaatctgtaccaactggaggggaacaaacggataacctgccgcaacggccaatggtccgagccacctaagtgcctgcatccatgtgtgatcagtcgggagatcatggagaactacaacattgccctgaggtggactgctaagcagaagctctatagccgaacaggcgagtcagtggagtttgtgtgtaaacggggatacaggctgtccagtaggagccacaccctgcgcactacttgctgggatgggaagctggaatatccaacttgc

SEQ ID NO: 22 - DNA, 2085 bp, synthetic construct
  source 1..2085: mol_type = other DNA
tgcggctctcctccacccattctcaatggaaggatctcctactacagcacccccatagctgtcggcaccgttatccgatacagttgttccggtactttccggcttatcggcgaaaagtctttgctgtgcattaccaaggataaagtggacgggacttgggacaaacccgcacctaagtgcgagtattttaacaaatatagcagctgccctgagcctatagtacccggggggtataaaatccggggctctactccctatcgtcatggcgattctgtgaccttcgcatgtaaaactaatttttcaatgaatggcaacaagtctgtatggtgtcaagcaaataacatgtggggacctacccgcctgccaacctgtgtgtcagtgtttcccctggaatgtccagccctccctatgatccacaacggacatcacaccagcgaaaacgttggctccatcgcaccagggctctctgtgacttactcttgcgagtccgggtacctgctcgtgggtgaaaagatcatcaactgcctcagtagtggtaaatggtccgccgtgcctcccacatgtgaagaggcccggtgcaagagcctgggccggttccccaacggaaaagtgaaggaacctcctatcttgagggttggtgtgaccgctaactttttctgcgacgaggggtacaggctccaagggcctccctctagtcggtgcgtaatcgccggtcaaggagtcgcatggactaagatgcctgtgtgtggcggaggtgggtcgggtggcggcggatctgaggactgcaacgaactgcctcctagaagaaacaccgaaatcctcacaggctcctggtcagatcagacctaccctgagggtacacaggccatctataaatgccgcccgggttaccgctccttgggcaatgttattatggtctgccggaaaggggaatgggtggccttgaaccccctcagaaagtgccaaaaaagaccctgcggacatccaggagacacacctttcgggacatttaccttgaccggtggtaacgtgttcgagtacggagtgaaggcagtctatacttgcaatgagggctaccagctcctgggggaaataaattatcgcgaatgtgatacagacggctggacgaacgacattcctatctgtgaggtggtcaaatgtctgcccgtcactgctcctgaaaacggcaagatagtgagttctgcaatggagccggatagggagtatcattttggtcaggccgtgcgctttgtgtgcaatagtgggtataaaatcgagggggatgaagaaatgcactgtagcgacgatggattctggtctaaagagaaacctaagtgtgtggagattagttgcaagagtccagacgtgattaacggtagccccatttcccaaaagataatatacaaggaaaacgaaagattccagtataaatgcaacatgggctacgagtatagcgagcggggcgatgccgtgtgtactgaaagcggctggcgccccctgccttcctgcgagattagggtgaagacctgttccaaaagcagcatcgacatcgaaaacggctttatatccgagagccagtatacgtatgcgctgaaggaaaaggccaagtatcagtgcaagctcggttatgtcacagctgatggcgagacctccgggtctatcacatgcggcaaagacggctggtccgctcagcctacctgcattaagagcgatagtacaggcaaatgtgggccacctcccccaattgataatggtgatataacctccttccctcttagtgtttacgccccagcatccagcgtggagtatcaatgccaaaatctgtaccaactggaggggaacaaacggataacctgccgcaacggccaatggtccgagccacctaagtgcctgcatccatgtgtgatcagtcgggagatcatggagaactacaacattgccctgaggtggactgctaagcagaagctctatagccgaacaggcgagtcagtggagtttgtgtgtaaacggggatacaggctgtccagtaggagccacaccctgcgcactacttgctgggatgggaagctggaatatccaacttgc

SEQ ID NO: 23 - DNA, 2172 bp, synthetic construct
  source 1..2172: mol_type = other DNA
atgccaatggggtccctacaacccctggcaacactatatctgctaggtatgctcgtggcctcctgtttaggaatttcatgcggctctcctccacccattctcaatggaaggatctcctactacagcacccccatagctgtcggcaccgttatccgatacagttgttccggtactttccggcttatcggcgaaaagtctttgctgtgcattaccaaggataaagtggacgggacttgggacaaacccgcacctaagtgcgagtattttaacaaatatagcagctgccctgagcctatagtacccggggggtataaaatccggggctctactccctatcgtcatggcgattctgtgaccttcgcatgtaaaactaatttttcaatgaatggcaacaagtctgtatggtgtcaagcaaataacatgtggggacctacccgcctgccaacctgtgtgtcagtgtttcccctggaatgtccagccctccctatgatccacaacggacatcacaccagcgaaaacgttggctccatcgcaccagggctctctgtgacttactcttgcgagtccgggtacctgctcgtgggtgaaaagatcatcaactgcctcagtagtggtaaatggtccgccgtgcctcccacatgtgaagaggcccggtgcaagagcctgggccggttccccaacggaaaagtgaaggaacctcctatcttgagggttggtgtgaccgctaactttttctgcgacgaggggtacaggctccaagggcctccctctagtcggtgcgtaatcgccggtcaaggagtcgcatggactaagatgcctgtgtgtggcggaggtgggtcgggtggcggcggatctgaggactgcaacgaactgcctcctagaagaaacaccgaaatcctcacaggctcctggtcagatcagacctaccctgagggtacacaggccatctataaatgccgcccgggttaccgctccttgggcaatgttattatggtctgccggaaaggggaatgggtggccttgaaccccctcagaaagtgccaaaaaagaccctgcggacatccaggagacacacctttcgggacatttaccttgaccggtggtaacgtgttcgagtacggagtgaaggcagtctatacttgcaatgagggctaccagctcctgggggaaataaattatcgcgaatgtgatacagacggctggacgaacgacattcctatctgtgaggtggtcaaatgtctgcccgtcactgctcctgaaaacggcaagatagtgagttctgcaatggagccggatagggagtatcattttggtcaggccgtgcgctttgtgtgcaatagtgggtataaaatcgagggggatgaagaaatgcactgtagcgacgatggattctggtctaaagagaaacctaagtgtgtggagattagttgcaagagtccagacgtgattaacggtagccccatttcccaaaagataatatacaaggaaaacgaaagattccagtataaatgcaacatgggctacgagtatagcgagcggggcgatgccgtgtgtactgaaagcggctggcgccccctgccttcctgcgagattagggtgaagacctgttccaaaagcagcatcgacatcgaaaacggctttatatccgagagccagtatacgtatgcgctgaaggaaaaggccaagtatcagtgcaagctcggttatgtcacagctgatggcgagacctccgggtctatcacatgcggcaaagacggctggtccgctcagcctacctgcattaagagcgatagtacaggcaaatgtgggccacctcccccaattgataatggtgatataacctccttccctcttagtgtttacgccccagcatccagcgtggagtatcaatgccaaaatctgtaccaactggaggggaacaaacggataacctgccgcaacggccaatggtccgagccacctaagtgcctgcatccatgtgtgatcagtcgggagatcatggagaactacaacattgccctgaggtggactgctaagcagaagctctatagccgaacaggcgagtcagtggagtttgtgtgtaaacggggatacaggctgtccagtaggagccacaccctgcgcactacttgctgggatgggaagctggaatatccaacttgcgccaagagg

SEQ ID NO: 24 - DNA, 543 bp, synthetic construct
  source 1..543: mol_type = other DNA
tgcgtgaaccctccaacagtccaaaatgcctatatagtctctaggcagatgagtaaatacccaagtggagagagagtgagataccagtgccggtctccttacgagatgttcggcgacgaggaagtgatgtgcctgaacggcaattggacagagccaccacaatgtaaggatagtacaggcaaatgtgggccacctcccccaattgataatggtgatataacctccttccctcttagtgtttacgccccagcatccagcgtggagtatcaatgccaaaatctgtaccaactggaggggaacaaacggataacctgccgcaacggccaatggtccgagccacctaagtgcctgcatccatgtgtgatcagtcgggagatcatggagaactacaacattgccctgaggtggactgctaagcagaagctctatagccgaacaggcgagtcagtggagtttgtgtgtaaacggggatacaggctgtccagtaggagccacaccctgcgcactacttgctgggatgggaagctggaatatccaacttgc

SEQ ID NO: 25 - DNA, 2067 bp, synthetic construct
  source 1..2067: mol_type = other DNA
tgcggctctcctccacccattctcaatggaaggatctcctactacagcacccccatagctgtcggcaccgttatccgatacagttgttccggtactttccggcttatcggcgaaaagtctttgctgtgcattaccaaggataaagtggacgggacttgggacaaacccgcacctaagtgcgagtattttaacaaatatagcagctgccctgagcctatagtacccggggggtataaaatccggggctctactccctatcgtcatggcgattctgtgaccttcgcatgtaaaactaatttttcaatgaatggcaacaagtctgtatggtgtcaagcaaataacatgtggggacctacccgcctgccaacctgtgtgtcagtgtttcccctggaatgtccagccctccctatgatccacaacggacatcacaccagcgaaaacgttggctccatcgcaccagggctctctgtgacttactcttgcgagtccgggtacctgctcgtgggtgaaaagatcatcaactgcctcagtagtggtaaatggtccgccgtgcctcccacatgtgaagaggcccggtgcaagagcctgggccggttccccaacggaaaagtgaaggaacctcctatcttgagggttggtgtgaccgctaactttttctgcgacgaggggtacaggctccaagggcctccctctagtcggtgcgtaatcgccggtcaaggagtcgcatggactaagatgcctgtgtgtggcggaggtgggtcgggtggcggcggatctgaggactgcaacgaactgcctcctagaagaaacaccgaaatcctcacaggctcctggtcagatcagacctaccctgagggtacacaggccatctataaatgccgcccgggttaccgctccttgggcaatgttattatggtctgccggaaaggggaatgggtggccttgaaccccctcagaaagtgccaaaaaagaccctgcggacatccaggagacacacctttcgggacatttaccttgaccggtggtaacgtgttcgagtacggagtgaaggcagtctatacttgcaatgagggctaccagctcctgggggaaataaattatcgcgaatgtgatacagacggctggacgaacgacattcctatctgtgaggtggtcaaatgtctgcccgtcactgctcctgaaaacggcaagatagtgagttctgcaatggagccggatagggagtatcattttggtcaggccgtgcgctttgtgtgcaatagtgggtataaaatcgagggggatgaagaaatgcactgtagcgacgatggattctggtctaaagagaaacctaagtgtgtggagattagttgcaagagtccagacgtgattaacggtagccccatttcccaaaagataatatacaaggaaaacgaaagattccagtataaatgcaacatgggctacgagtatagcgagcggggcgatgccgtgtgtactgaaagcggctggcgccccctgccttcctgcgagcgggatacaagctgcgtgaaccctccaacagtccaaaatgcctatatagtctctaggcagatgagtaaatacccaagtggagagagagtgagataccagtgccggtctccttacgagatgttcggcgacgaggaagtgatgtgcctgaacggcaattggacagagccaccacaatgtaaggatagtacaggcaaatgtgggccacctcccccaattgataatggtgatataacctccttccctcttagtgtttacgccccagcatccagcgtggagtatcaatgccaaaatctgtaccaactggaggggaacaaacggataacctgccgcaacggccaatggtccgagccacctaagtgcctgcatccatgtgtgatcagtcgggagatcatggagaactacaacattgccctgaggtggactgctaagcagaagctctatagccgaacaggcgagtcagtggagtttgtgtgtaaacggggatacaggctgtccagtaggagccacaccctgcgcactacttgctgggatgggaagctggaatatccaacttgc

SEQ ID NO: 26 - DNA, 2154 bp, synthetic construct
  source 1..2154: mol_type = other DNA
atgccaatggggtccctacaacccctggcaacactatatctgctaggtatgctcgtggcctcctgtttaggaatttcatgcggctctcctccacccattctcaatggaaggatctcctactacagcacccccatagctgtcggcaccgttatccgatacagttgttccggtactttccggcttatcggcgaaaagtctttgctgtgcattaccaaggataaagtggacgggacttgggacaaacccgcacctaagtgcgagtattttaacaaatatagcagctgccctgagcctatagtacccggggggtataaaatccggggctctactccctatcgtcatggcgattctgtgaccttcgcatgtaaaactaatttttcaatgaatggcaacaagtctgtatggtgtcaagcaaataacatgtggggacctacccgcctgccaacctgtgtgtcagtgtttcccctggaatgtccagccctccctatgatccacaacggacatcacaccagcgaaaacgttggctccatcgcaccagggctctctgtgacttactcttgcgagtccgggtacctgctcgtgggtgaaaagatcatcaactgcctcagtagtggtaaatggtccgccgtgcctcccacatgtgaagaggcccggtgcaagagcctgggccggttccccaacggaaaagtgaaggaacctcctatcttgagggttggtgtgaccgctaactttttctgcgacgaggggtacaggctccaagggcctccctctagtcggtgcgtaatcgccggtcaaggagtcgcatggactaagatgcctgtgtgtggcggaggtgggtcgggtggcggcggatctgaggactgcaacgaactgcctcctagaagaaacaccgaaatcctcacaggctcctggtcagatcagacctaccctgagggtacacaggccatctataaatgccgcccgggttaccgctccttgggcaatgttattatggtctgccggaaaggggaatgggtggccttgaaccccctcagaaagtgccaaaaaagaccctgcggacatccaggagacacacctttcgggacatttaccttgaccggtggtaacgtgttcgagtacggagtgaaggcagtctatacttgcaatgagggctaccagctcctgggggaaataaattatcgcgaatgtgatacagacggctggacgaacgacattcctatctgtgaggtggtcaaatgtctgcccgtcactgctcctgaaaacggcaagatagtgagttctgcaatggagccggatagggagtatcattttggtcaggccgtgcgctttgtgtgcaatagtgggtataaaatcgagggggatgaagaaatgcactgtagcgacgatggattctggtctaaagagaaacctaagtgtgtggagattagttgcaagagtccagacgtgattaacggtagccccatttcccaaaagataatatacaaggaaaacgaaagattccagtataaatgcaacatgggctacgagtatagcgagcggggcgatgccgtgtgtactgaaagcggctggcgccccctgccttcctgcgagcgggatacaagctgcgtgaaccctccaacagtccaaaatgcctatatagtctctaggcagatgagtaaatacccaagtggagagagagtgagataccagtgccggtctccttacgagatgttcggcgacgaggaagtgatgtgcctgaacggcaattggacagagccaccacaatgtaaggatagtacaggcaaatgtgggccacctcccccaattgataatggtgatataacctccttccctcttagtgtttacgccccagcatccagcgtggagtatcaatgccaaaatctgtaccaactggaggggaacaaacggataacctgccgcaacggccaatggtccgagccacctaagtgcctgcatccatgtgtgatcagtcgggagatcatggagaactacaacattgccctgaggtggactgctaagcagaagctctatagccgaacaggcgagtcagtggagtttgtgtgtaaacggggatacaggctgtccagtaggagccacaccctgcgcactacttgctgggatgggaagctggaatatccaacttgcgccaagagg

SEQ ID NO: 27 - DNA, 747 bp, synthetic construct
  source 1..747: mol_type = other DNA
tgcggcagcccccctcccatcctgaacggcagaatcagctactacagcacccccatcgccgtgggcaccgtgatcagatacagctgcagcggcaccttcagactgatcggcgagaagagcctgctgtgcatcaccaaggacaaggtggacggcacctgggacaagcccgcccccaagtgcgagtacttcaacaagtacagcagctgccccgagcccatcgtgcctggcggctacaagatcagaggcagcaccccctacagacacggcgacagcgtgaccttcgcctgcaagaccaacttcagcatgaacggcaacaagagcgtgtggtgccaagccaacaacatgtggggccccacaagactgcccacctgcgtgagcgtgttccccctggagtgccccgccctgcccatgatccacaacggccaccacacaagcgagaacgtgggcagcatcgcccccggcctgagcgtgacctacagctgcgagagcggctacctgctggtgggcgagaagatcatcaactgcctgagcagcggcaagtggagcgccgtgccccccacctgcgaggaggctagatgcaagagcctgggcagattccccaacggcaaggtgaaggagcctcctatcctgagagtgggcgtgaccgccaacttcttctgcgacgagggctacagactgcaaggcccccctagcagcagatgtgtgatcgctggccaaggcgtggcctggaccaaaatgcccgtctgc

SEQ ID NO: 28 - DNA, 726 bp, synthetic construct
  source 1..726: mol_type = other DNA
tgcaacgagctgccccctagacggaacacagagatcctgaccggcagctggagcgatcaaacatatcccgagggcacccaagccatctacaaatgcagacctggctacagaagcctgggcaatgtgatcatggtctgccggaaaggggagtgggtcgctctgaaccccctgcggaagtgtcagaagagaccttgcggccaccccggcgacacacccttcgggaccttcacactgaccggcggcaacgtgtttgagtacggcgtcaaggccgtgtacacctgtaacgaggggtatcagctgctgggcgagatcaactacagagagtgcgataccgacggctggaccaatgacatccccatctgcgaggtggtgaagtgtctgcccgtgaccgcccccgaaaacggcaagatcgtgagcagcgccatggagcccgaccgggagtaccattttgggcaagctgtgagattcgtctgcaatagcggctacaagatcgaaggcgacgaggagatgcactgtagcgacgacggcttctggtccaaagagaaacccaaatgcgtggagatctcctgcaaaagccccgatgtgatcaacggcagccccatctcccaaaaaattatctacaaggaaaacgaacggtttcagtacaaatgcaacatgggctacgaatactccgagcggggggatgccgtgtgcaccgagagcggctggcggcctctgcctagctgt

SEQ ID NO: 29 - DNA, 726 bp, synthetic construct
  source 1..726: mol_type = other DNA
tgcaatgaactgcctcctagacggaacaccgaaatcctgaccgggagctggagcgaccaaacataccccgaggggacacaagccatctacaagtgcagacctgggtatagatccctcgggaacgtgatcatggtctgtcggaagggcgagtgggtcgctctgaaccctctcagaaagtgtcagaaacggccctgcgggcaccccggcgatacccccttcggcacattcaccctgaccggggggaacgtgttcgagtacggcgtgaaggccgtctacacctgcaacgagggctaccaactcctgggcgaaatcaattacagagaatgcgacacagatggctggaccaacgacatccctatctgcgaggtcgtgaaatgtctccccgtgacagcccctgagaacggcaagattgtcagcagcgctatggaacctgatagagagtaccatttcggccaagccgtcagatttgtgtgcaattccggctacaaaattgagggggacgaagagatgcactgctccgacgatggcttctggagcaaggaaaaacccaagtgcgtggagattagctgcaagagccccgacgtgatcaacgggagccccatctcccaaaaaatcatctacaaggagaacgagagatttcagtataagtgcaacatgggctatgagtacagcgagcggggggacgccgtgtgtaccgaatccgggtggagacccctgcctagctgc

SEQ ID NO: 30 - DNA, 2274 bp, synthetic construct
  source 1..2274: mol_type = other DNA
tgcggcagcccccctcccatcctgaacggcagaatcagctactacagcacccccatcgccgtgggcaccgtgatcagatacagctgcagcggcaccttcagactgatcggcgagaagagcctgctgtgcatcaccaaggacaaggtggacggcacctgggacaagcccgcccccaagtgcgagtacttcaacaagtacagcagctgccccgagcccatcgtgcctggcggctacaagatcagaggcagcaccccctacagacacggcgacagcgtgaccttcgcctgcaagaccaacttcagcatgaacggcaacaagagcgtgtggtgccaagccaacaacatgtggggccccacaagactgcccacctgcgtgagcgtgttccccctggagtgccccgccctgcccatgatccacaacggccaccacacaagcgagaacgtgggcagcatcgcccccggcctgagcgtgacctacagctgcgagagcggctacctgctggtgggcgagaagatcatcaactgcctgagcagcggcaagtggagcgccgtgccccccacctgcgaggaggctagatgcaagagcctgggcagattccccaacggcaaggtgaaggagcctcctatcctgagagtgggcgtgaccgccaacttcttctgcgacgagggctacagactgcaaggcccccctagcagcagatgtgtgatcgctggccaaggcgtggcctggaccaaaatgcccgtctgcgggggggggggcagcgggggcgggggcagcgaggattgcaacgagctgccccctagacggaacacagagatcctgaccggcagctggagcgatcaaacatatcccgagggcacccaagccatctacaaatgcagacctggctacagaagcctgggcaatgtgatcatggtctgccggaaaggggagtgggtcgctctgaaccccctgcggaagtgtcagaagagaccttgcggccaccccggcgacacacccttcgggaccttcacactgaccggcggcaacgtgtttgagtacggcgtcaaggccgtgtacacctgtaacgaggggtatcagctgctgggcgagatcaactacagagagtgcgataccgacggctggaccaatgacatccccatctgcgaggtggtgaagtgtctgcccgtgaccgcccccgaaaacggcaagatcgtgagcagcgccatggagcccgaccgggagtaccattttgggcaagctgtgagattcgtctgcaatagcggctacaagatcgaaggcgacgaggagatgcactgtagcgacgacggcttctggtccaaagagaaacccaaatgcgtggagatctcctgcaaaagccccgatgtgatcaacggcagccccatctcccaaaaaattatctacaaggaaaacgaacggtttcagtacaaatgcaacatgggctacgaatactccgagcggggggatgccgtgtgcaccgagagcggctggcggcctctgcctagctgtgaagggggcggcgggagcggcgggggcggcagcgaggactgcaatgaactgcctcctagacggaacaccgaaatcctgaccgggagctggagcgaccaaacataccccgaggggacacaagccatctacaagtgcagacctgggtatagatccctcgggaacgtgatcatggtctgtcggaagggcgagtgggtcgctctgaaccctctcagaaagtgtcagaaacggccctgcgggcaccccggcgatacccccttcggcacattcaccctgaccggggggaacgtgttcgagtacggcgtgaaggccgtctacacctgcaacgagggctaccaactcctgggcgaaatcaattacagagaatgcgacacagatggctggaccaacgacatccctatctgcgaggtcgtgaaatgtctccccgtgacagcccctgagaacggcaagattgtcagcagcgctatggaacctgatagagagtaccatttcggccaagccgtcagatttgtgtgcaattccggctacaaaattgagggggacgaagagatgcactgctccgacgatggcttctggagcaaggaaaaacccaagtgcgtggagattagctgcaagagccccgacgtgatcaacgggagccccatctcccaaaaaatcatctacaaggagaacgagagatttcagtataagtgcaacatgggctatgagtacagcgagcggggggacgccgtgtgtaccgaatccgggtggagacccctgcctagctgc

SEQ ID NO: 31 - DNA, 2355 bp, synthetic construct
  source 1..2355: mol_type = other DNA
atgcccatgggcagcctgcagcccctggccaccctgtacctgctgggcatgctggtggctagctgcctgggcatcagctgcggcagcccccctcccatcctgaacggcagaatcagctactacagcacccccatcgccgtgggcaccgtgatcagatacagctgcagcggcaccttcagactgatcggcgagaagagcctgctgtgcatcaccaaggacaaggtggacggcacctgggacaagcccgcccccaagtgcgagtacttcaacaagtacagcagctgccccgagcccatcgtgcctggcggctacaagatcagaggcagcaccccctacagacacggcgacagcgtgaccttcgcctgcaagaccaacttcagcatgaacggcaacaagagcgtgtggtgccaagccaacaacatgtggggccccacaagactgcccacctgcgtgagcgtgttccccctggagtgccccgccctgcccatgatccacaacggccaccacacaagcgagaacgtgggcagcatcgcccccggcctgagcgtgacctacagctgcgagagcggctacctgctggtgggcgagaagatcatcaactgcctgagcagcggcaagtggagcgccgtgccccccacctgcgaggaggctagatgcaagagcctgggcagattccccaacggcaaggtgaaggagcctcctatcctgagagtgggcgtgaccgccaacttcttctgcgacgagggctacagactgcaaggcccccctagcagcagatgtgtgatcgctggccaaggcgtggcctggaccaaaatgcccgtctgcgggggggggggcagcgggggcgggggcagcgaggattgcaacgagctgccccctagacggaacacagagatcctgaccggcagctggagcgatcaaacatatcccgagggcacccaagccatctacaaatgcagacctggctacagaagcctgggcaatgtgatcatggtctgccggaaaggggagtgggtcgctctgaaccccctgcggaagtgtcagaagagaccttgcggccaccccggcgacacacccttcgggaccttcacactgaccggcggcaacgtgtttgagtacggcgtcaaggccgtgtacacctgtaacgaggggtatcagctgctgggcgagatcaactacagagagtgcgataccgacggctggaccaatgacatccccatctgcgaggtggtgaagtgtctgcccgtgaccgcccccgaaaacggcaagatcgtgagcagcgccatggagcccgaccgggagtaccattttgggcaagctgtgagattcgtctgcaatagcggctacaagatcgaaggcgacgaggagatgcactgtagcgacgacggcttctggtccaaagagaaacccaaatgcgtggagatctcctgcaaaagccccgatgtgatcaacggcagccccatctcccaaaaaattatctacaaggaaaacgaacggtttcagtacaaatgcaacatgggctacgaatactccgagcggggggatgccgtgtgcaccgagagcggctggcggcctctgcctagctgtgaagggggcggcgggagcggcgggggcggcagcgaggactgcaatgaactgcctcctagacggaacaccgaaatcctgaccgggagctggagcgaccaaacataccccgaggggacacaagccatctacaagtgcagacctgggtatagatccctcgggaacgtgatcatggtctgtcggaagggcgagtgggtcgctctgaaccctctcagaaagtgtcagaaacggccctgcgggcaccccggcgatacccccttcggcacattcaccctgaccggggggaacgtgttcgagtacggcgtgaaggccgtctacacctgcaacgagggctaccaactcctgggcgaaatcaattacagagaatgcgacacagatggctggaccaacgacatccctatctgcgaggtcgtgaaatgtctccccgtgacagcccctgagaacggcaagattgtcagcagcgctatggaacctgatagagagtaccatttcggccaagccgtcagatttgtgtgcaattccggctacaaaattgagggggacgaagagatgcactgctccgacgatggcttctggagcaaggaaaaacccaagtgcgtggagattagctgcaagagccccgacgtgatcaacgggagccccatctcccaaaaaatcatctacaaggagaacgagagatttcagtataagtgcaacatgggctatgagtacagcgagcggggggacgccgtgtgtaccgaatccgggtggagacccctgcctagctgcgag

SEQ ID NO: 32 - DNA, 1509 bp, synthetic construct
  source 1..1509: mol_type = other DNA
tgcggctctcctccacccattctcaatggaaggatctcctactacagcacccccatagctgtcggcaccgttatccgatacagttgttccggtactttccggcttatcggcgaaaagtctttgctgtgcattaccaaggataaagtggacgggacttgggacaaacccgcacctaagtgcgagtattttaacaaatatagcagctgccctgagcctatagtacccggggggtataaaatccggggctctactccctatcgtcatggcgattctgtgaccttcgcatgtaaaactaatttttcaatgaatggcaacaagtctgtatggtgtcaagcaaataacatgtggggacctacccgcctgccaacctgtgtgtcagtgtttcccctggaatgtccagccctccctatgatccacaacggacatcacaccagcgaaaacgttggctccatcgcaccagggctctctgtgacttactcttgcgagtccgggtacctgctcgtgggtgaaaagatcatcaactgcctcagtagtggtaaatggtccgccgtgcctcccacatgtgaagaggcccggtgcaagagcctgggccggttccccaacggaaaagtgaaggaacctcctatcttgagggttggtgtgaccgctaactttttctgcgacgaggggtacaggctccaagggcctccctctagtcggtgcgtaatcgccggtcaaggagtcgcatggactaagatgcctgtgtgtggcggaggtgggtcgggtggcggcggatctgaagactgtaatgagctgcccccaagacggaatacagagatcctcacaggctcttggtccgatcaaacttatccagagggtacccaggcaatttacaagtgcagacctggatacaggagcctgggcaatgtgattatggtgtgccgcaagggggagtgggtggcccttaatcctctccggaagtgtcagaaaagaccatgcggacaccctggagatacacctttcggtacctttacccttaccggcggcaatgtcttcgagtatggcgtcaaggccgtgtacacttgtaacgagggataccagctgctgggggaaataaactatcgtgagtgtgacactgacgggtggactaacgacatccccatttgcgaggtggtcaagtgccttcctgtaaccgctcccgaaaatggtaagatcgtatcttccgcaatggagcctgatcgggaataccactttggacaagccgttcggttcgtatgtaattcagggtataaaattgagggcgatgaggagatgcactgcagtgatgacggcttttggtcaaaggaaaagccaaagtgcgtagagatcagttgtaagtctcctgacgttattaacgggagtcccatcagtcagaagatcatttacaaggaaaacgagaggttccagtataaatgcaatatgggatatgagtactccgaaagaggggacgccgtgtgcacagagtccggatggcgacctttgccatcttgt

SEQ ID NO: 33 - DNA, 1590 bp, synthetic construct
  source 1..1590: mol_type = other DNA
atgccaatggggtccctacaacccctggcaacactatatctgctaggtatgctcgtggcctcctgtttaggaatttcatgcggctctcctccacccattctcaatggaaggatctcctactacagcacccccatagctgtcggcaccgttatccgatacagttgttccggtactttccggcttatcggcgaaaagtctttgctgtgcattaccaaggataaagtggacgggacttgggacaaacccgcacctaagtgcgagtattttaacaaatatagcagctgccctgagcctatagtacccggggggtataaaatccggggctctactccctatcgtcatggcgattctgtgaccttcgcatgtaaaactaatttttcaatgaatggcaacaagtctgtatggtgtcaagcaaataacatgtggggacctacccgcctgccaacctgtgtgtcagtgtttcccctggaatgtccagccctccctatgatccacaacggacatcacaccagcgaaaacgttggctccatcgcaccagggctctctgtgacttactcttgcgagtccgggtacctgctcgtgggtgaaaagatcatcaactgcctcagtagtggtaaatggtccgccgtgcctcccacatgtgaagaggcccggtgcaagagcctgggccggttccccaacggaaaagtgaaggaacctcctatcttgagggttggtgtgaccgctaactttttctgcgacgaggggtacaggctccaagggcctccctctagtcggtgcgtaatcgccggtcaaggagtcgcatggactaagatgcctgtgtgtggcggaggtgggtcgggtggcggcggatctgaagactgtaatgagctgcccccaagacggaatacagagatcctcacaggctcttggtccgatcaaacttatccagagggtacccaggcaatttacaagtgcagacctggatacaggagcctgggcaatgtgattatggtgtgccgcaagggggagtgggtggcccttaatcctctccggaagtgtcagaaaagaccatgcggacaccctggagatacacctttcggtacctttacccttaccggcggcaatgtcttcgagtatggcgtcaaggccgtgtacacttgtaacgagggataccagctgctgggggaaataaactatcgtgagtgtgacactgacgggtggactaacgacatccccatttgcgaggtggtcaagtgccttcctgtaaccgctcccgaaaatggtaagatcgtatcttccgcaatggagcctgatcgggaataccactttggacaagccgttcggttcgtatgtaattcagggtataaaattgagggcgatgaggagatgcactgcagtgatgacggcttttggtcaaaggaaaagccaaagtgcgtagagatcagttgtaagtctcctgacgttattaacgggagtcccatcagtcagaagatcatttacaaggaaaacgagaggttccagtataaatgcaatatgggatatgagtactccgaaagaggggacgccgtgtgcacagagtccggatggcgacctttgccatcttgtgaa

SEQ ID NO: 34 - DNA, 900 bp, synthetic construct
  source 1..900: mol_type = other DNA
tgtaatgagctgcccccaagacggaatacagagatcctcacaggctcttggtccgatcaaacttatccagagggtacccaggcaatttacaagtgcagacctggatacaggagcctgggcaatgtgattatggtgtgccgcaagggggagtgggtggcccttaatcctctccggaagtgtcagaaaagaccatgcggacaccctggagatacacctttcggtacctttacccttaccggcggcaatgtcttcgagtatggcgtcaaggccgtgtacacttgtaacgagggataccagctgctgggggaaataaactatcgtgagtgtgacactgacgggtggactaacgacatccccatttgcgaggtggtcaagtgccttcctgtaaccgctcccgaaaatggtaagatcgtatcttccgcaatggagcctgatcgggaataccactttggacaagccgttcggttcgtatgtaattcagggtataaaattgagggcgatgaggagatgcactgcagtgatgacggcttttggtcaaaggaaaagccaaagtgcgtagagatcagttgtaagtctcctgacgttattaacgggagtcccatcagtcagaagatcatttacaaggaaaacgagaggttccagtataaatgcaatatgggatatgagtactccgaaagaggggacgccgtgtgcacagagtccggatggcgacctttgccatcttgtgaagaaaagtcttgtgacaacccctatattcctaacggagattactctcctctgcgcatcaagcaccgaactggggacgagatcacttaccaatgtcgaaacggcttctaccctgctaccagaggtaacactgccaagtgtaccagcaccggttggattcccgcccccagatgc

SEQ ID NO: 35 - DNA, 1683 bp, synthetic construct
  source 1..1683: mol_type = other DNA
tgcggctctcctccacccattctcaatggaaggatctcctactacagcacccccatagctgtcggcaccgttatccgatacagttgttccggtactttccggcttatcggcgaaaagtctttgctgtgcattaccaaggataaagtggacgggacttgggacaaacccgcacctaagtgcgagtattttaacaaatatagcagctgccctgagcctatagtacccggggggtataaaatccggggctctactccctatcgtcatggcgattctgtgaccttcgcatgtaaaactaatttttcaatgaatggcaacaagtctgtatggtgtcaagcaaataacatgtggggacctacccgcctgccaacctgtgtgtcagtgtttcccctggaatgtccagccctccctatgatccacaacggacatcacaccagcgaaaacgttggctccatcgcaccagggctctctgtgacttactcttgcgagtccgggtacctgctcgtgggtgaaaagatcatcaactgcctcagtagtggtaaatggtccgccgtgcctcccacatgtgaagaggcccggtgcaagagcctgggccggttccccaacggaaaagtgaaggaacctcctatcttgagggttggtgtgaccgctaactttttctgcgacgaggggtacaggctccaagggcctccctctagtcggtgcgtaatcgccggtcaaggagtcgcatggactaagatgcctgtgtgtggcggaggtgggtcgggtggcggcggatctgaagactgtaatgagctgcccccaagacggaatacagagatcctcacaggctcttggtccgatcaaacttatccagagggtacccaggcaatttacaagtgcagacctggatacaggagcctgggcaatgtgattatggtgtgccgcaagggggagtgggtggcccttaatcctctccggaagtgtcagaaaagaccatgcggacaccctggagatacacctttcggtacctttacccttaccggcggcaatgtcttcgagtatggcgtcaaggccgtgtacacttgtaacgagggataccagctgctgggggaaataaactatcgtgagtgtgacactgacgggtggactaacgacatccccatttgcgaggtggtcaagtgccttcctgtaaccgctcccgaaaatggtaagatcgtatcttccgcaatggagcctgatcgggaataccactttggacaagccgttcggttcgtatgtaattcagggtataaaattgagggcgatgaggagatgcactgcagtgatgacggcttttggtcaaaggaaaagccaaagtgcgtagagatcagttgtaagtctcctgacgttattaacgggagtcccatcagtcagaagatcatttacaaggaaaacgagaggttccagtataaatgcaatatgggatatgagtactccgaaagaggggacgccgtgtgcacagagtccggatggcgacctttgccatcttgtgaagaaaagtcttgtgacaacccctatattcctaacggagattactctcctctgcgcatcaagcaccgaactggggacgagatcacttaccaatgtcgaaacggcttctaccctgctaccagaggtaacactgccaagtgtaccagcaccggttggattcccgcccccagatgc

SEQ ID NO: 36 - DNA, 1770 bp, synthetic construct
  source 1..1770: mol_type = other DNA
atgccaatggggtccctacaacccctggcaacactatatctgctaggtatgctcgtggcctcctgtttaggaatttcatgcggctctcctccacccattctcaatggaaggatctcctactacagcacccccatagctgtcggcaccgttatccgatacagttgttccggtactttccggcttatcggcgaaaagtctttgctgtgcattaccaaggataaagtggacgggacttgggacaaacccgcacctaagtgcgagtattttaacaaatatagcagctgccctgagcctatagtacccggggggtataaaatccggggctctactccctatcgtcatggcgattctgtgaccttcgcatgtaaaactaatttttcaatgaatggcaacaagtctgtatggtgtcaagcaaataacatgtggggacctacccgcctgccaacctgtgtgtcagtgtttcccctggaatgtccagccctccctatgatccacaacggacatcacaccagcgaaaacgttggctccatcgcaccagggctctctgtgacttactcttgcgagtccgggtacctgctcgtgggtgaaaagatcatcaactgcctcagtagtggtaaatggtccgccgtgcctcccacatgtgaagaggcccggtgcaagagcctgggccggttccccaacggaaaagtgaaggaacctcctatcttgagggttggtgtgaccgctaactttttctgcgacgaggggtacaggctccaagggcctccctctagtcggtgcgtaatcgccggtcaaggagtcgcatggactaagatgcctgtgtgtggcggaggtgggtcgggtggcggcggatctgaagactgtaatgagctgcccccaagacggaatacagagatcctcacaggctcttggtccgatcaaacttatccagagggtacccaggcaatttacaagtgcagacctggatacaggagcctgggcaatgtgattatggtgtgccgcaagggggagtgggtggcccttaatcctctccggaagtgtcagaaaagaccatgcggacaccctggagatacacctttcggtacctttacccttaccggcggcaatgtcttcgagtatggcgtcaaggccgtgtacacttgtaacgagggataccagctgctgggggaaataaactatcgtgagtgtgacactgacgggtggactaacgacatccccatttgcgaggtggtcaagtgccttcctgtaaccgctcccgaaaatggtaagatcgtatcttccgcaatggagcctgatcgggaataccactttggacaagccgttcggttcgtatgtaattcagggtataaaattgagggcgatgaggagatgcactgcagtgatgacggcttttggtcaaaggaaaagccaaagtgcgtagagatcagttgtaagtctcctgacgttattaacgggagtcccatcagtcagaagatcatttacaaggaaaacgagaggttccagtataaatgcaatatgggatatgagtactccgaaagaggggacgccgtgtgcacagagtccggatggcgacctttgccatcttgtgaagaaaagtcttgtgacaacccctatattcctaacggagattactctcctctgcgcatcaagcaccgaactggggacgagatcacttaccaatgtcgaaacggcttctaccctgctaccagaggtaacactgccaagtgtaccagcaccggttggattcccgcccccagatgcacacttaaa

SEQ ID NO: 37 - DNA, 72 bp, synthetic construct
  source 1..72: mol_type = other DNA
atgccaatggggtccctacaacccctggcaacactatatctgctaggtatgctcgtggcctcctgtttagga

SEQ ID NO: 38 - DNA, 72 bp, synthetic construct
  source 1..72: mol_type = other DNA
atgcccatgggcagcctgcagcccctggccaccctgtacctgctgggcatgctggtggctagctgcctgggc

SEQ ID NO: 39 - protein, 55 aa, synthetic construct
CVNPPTVQNAYIVSRQMSKYPSGERVRYQCRSPYEMFGDEEVMCLNGNWTEPPQC

SEQ ID NO: 40 - protein, 62 aa, synthetic construct
CVISREIMENYNIALRWTAKQKLYSRTGESVEFVCKRGYRLSSRSHTLRTTCWDGKLEYPTC

SEQ ID NO: 41 - protein, 631 aa, synthetic construct
CGSPPPILNGRISYYSTPIAVGTVIRYSCSGTFRLIGEKSLLCITKDKVDGTWDKPAPKCEYFNKYSSCPEPIVPGGYKIRGSTPYRHGDSVTFACKTNFSMNGNKSVWCQANNMWGPTRLPTCVSVFPLECPALPMIHNGHHTSENVGSIAPGLSVTYSCESGYLLVGEKIINCLSSGKWSAVPPTCEEARCKSLGRFPNGKVKEPPILRVGVTANFFCDEGYRLQGPPSSRCVIAGQGVAWTKMPVCGGGGSGGGGSEDCNELPPRRNTEILTGSWSDQTYPEGTQAIYKCRPGYRSLGNVIMVCRKGEWVALNPLRKCQKRPCGHPGDTPFGTFTLTGGNVFEYGVKAVYTCNEGYQLLGEINYRECDTDGWTNDIPICEVVKCLPVTAPENGKIVSSAMEPDREYHFGQAVRFVCNSGYKIEGDEEMHCSDDGFWSKEKPKCVEISCKSPDVINGSPISQKIIYKENERFQYKCNMGYEYSERGDAVCTESGWRPLPSCERDTSCVNPPTVQNAYIVSRQMSKYPSGERVRYQCRSPYEMFGDEEVMCLNGNWTEPPQCKDSTGKCVISREIMENYNIALRWTAKQKLYSRTGESVEFVCKRGYRLSSRSHTLRTTCWDGKLEYPTC

SEQ ID NO: 42 - protein, 660 aa, synthetic construct
MPMGSLQPLATLYLLGMLVASCLGISCGSPPPILNGRISYYSTPIAVGTVIRYSCSGTFRLIGEKSLLCITKDKVDGTWDKPAPKCEYFNKYSSCPEPIVPGGYKIRGSTPYRHGDSVTFACKTNFSMNGNKSVWCQANNMWGPTRLPTCVSVFPLECPALPMIHNGHHTSENVGSIAPGLSVTYSCESGYLLVGEKIINCLSSGKWSAVPPTCEEARCKSLGRFPNGKVKEPPILRVGVTANFFCDEGYRLQGPPSSRCVIAGQGVAWTKMPVCGGGGSGGGGSEDCNELPPRRNTEILTGSWSDQTYPEGTQAIYKCRPGYRSLGNVIMVCRKGEWVALNPLRKCQKRPCGHPGDTPFGTFTLTGGNVFEYGVKAVYTCNEGYQLLGEINYRECDTDGWTNDIPICEVVKCLPVTAPENGKIVSSAMEPDREYHFGQAVRFVCNSGYKIEGDEEMHCSDDGFWSKEKPKCVEISCKSPDVINGSPISQKIIYKENERFQYKCNMGYEYSERGDAVCTESGWRPLPSCERDTSCVNPPTVQNAYIVSRQMSKYPSGERVRYQCRSPYEMFGDEEVMCLNGNWTEPPQCKDSTGKCVISREIMENYNIALRWTAKQKLYSRTGESVEFVCKRGYRLSSRSHTLRTTCWDGKLEYPTCAKR

SEQ ID NO: 43 - protein, 54 aa, synthetic construct
CYFPYLENGYNQNHGRKFVQGKSIDVACHPGYALPKAQTTVTCMENGWSPTPRC

SEQ ID NO: 44 - protein, 826 aa, synthetic construct
CGSPPPILNGRISYYSTPIAVGTVIRYSCSGTFRLIGEKSLLCITKDKVDGTWDKPAPKCEYFNKYSSCPEPIVPGGYKIRGSTPYRHGDSVTFACKTNFSMNGNKSVWCQANNMWGPTRLPTCVSVFPLECPALPMIHNGHHTSENVGSIAPGLSVTYSCESGYLLVGEKIINCLSSGKWSAVPPTCEEARCKSLGRFPNGKVKEPPILRVGVTANFFCDEGYRLQGPPSSRCVIAGQGVAWTKMPVCGGGGSGGGGSEDCNELPPRRNTEILTGSWSDQTYPEGTQAIYKCRPGYRSLGNVIMVCRKGEWVALNPLRKCQKRPCGHPGDTPFGTFTLTGGNVFEYGVKAVYTCNEGYQLLGEINYRECDTDGWTNDIPICEVVKCLPVTAPENGKIVSSAMEPDREYHFGQAVRFVCNSGYKIEGDEEMHCSDDGFWSKEKPKCVEISCKSPDVINGSPISQKIIYKENERFQYKCNMGYEYSERGDAVCTESGWRPLPSCEGGGGSGGGGSEDCNELPPRRNTEILTGSWSDQTYPEGTQAIYKCRPGYRSLGNVIMVCRKGEWVALNPLRKCQKRPCGHPGDTPFGTFTLTGGNVFEYGVKAVYTCNEGYQLLGEINYRECDTDGWTNDIPICEVVKCLPVTAPENGKIVSSAMEPDREYHFGQAVRFVCNSGYKIEGDEEMHCSDDGFWSKEKPKCVEISCKSPDVINGSPISQKIIYKENERFQYKCNMGYEYSERGDAVCTESGWRPLPSCEGGGGSGGGGSLRKCYFPYLENGYNQNHGRKFVQGKSIDVACHPGYALPKAQTTVTCMENGWSPTPRC

SEQ ID NO: 45 - protein, 858 aa, synthetic construct
MPMGSLQPLATLYLLGMLVASCLGISCGSPPPILNGRISYYSTPIAVGTVIRYSCSGTFRLIGEKSLLCITKDKVDGTWDKPAPKCEYFNKYSSCPEPIVPGGYKIRGSTPYRHGDSVTFACKTNFSMNGNKSVWCQANNMWGPTRLPTCVSVFPLECPALPMIHNGHHTSENVGSIAPGLSVTYSCESGYLLVGEKIINCLSSGKWSAVPPTCEEARCKSLGRFPNGKVKEPPILRVGVTANFFCDEGYRLQGPPSSRCVIAGQGVAWTKMPVCGGGGSGGGGSEDCNELPPRRNTEILTGSWSDQTYPEGTQAIYKCRPGYRSLGNVIMVCRKGEWVALNPLRKCQKRPCGHPGDTPFGTFTLTGGNVFEYGVKAVYTCNEGYQLLGEINYRECDTDGWTNDIPICEVVKCLPVTAPENGKIVSSAMEPDREYHFGQAVRFVCNSGYKIEGDEEMHCSDDGFWSKEKPKCVEISCKSPDVINGSPISQKIIYKENERFQYKCNMGYEYSERGDAVCTESGWRPLPSCEGGGGSGGGGSEDCNELPPRRNTEILTGSWSDQTYPEGTQAIYKCRPGYRSLGNVIMVCRKGEWVALNPLRKCQKRPCGHPGDTPFGTFTLTGGNVFEYGVKAVYTCNEGYQLLGEINYRECDTDGWTNDIPICEVVKCLPVTAPENGKIVSSAMEPDREYHFGQAVRFVCNSGYKIEGDEEMHCSDDGFWSKEKPKCVEISCKSPDVINGSPISQKIIYKENERFQYKCNMGYEYSERGDAVCTESGWRPLPSCEGGGGSGGGGSLRKCYFPYLENGYNQNHGRKFVQGKSIDVACHPGYALPKAQTTVTCMENGWSPTPRCIRVKTY

SEQ ID NO: 46 - protein, 249 aa, synthetic construct
CGSPPPILNGRISYYSTPIAVGTVIRYSCSGTFALIGEASLLCITKDKVDGTWDKPAPKCEYFNAYSSCPEPIVPGGYKIRGSTPYRHGDSVTFACKTNFSMNGNKSVWCQANNMWGPTRLPTCVSVFPLECPALPMIHNGHHTSENVGSIAPGLSVTYSCESGYLLVGEKIINCLSSGKWSAVPPTCEEARCKSLGRFPNGKVKEPPILRVGVTANFFCDEGYRLQGPPSSRCVIAGQGVAWTKMPVC

SEQ ID NO: 47 - protein, 695 aa, synthetic construct
CGSPPPILNGRISYYSTPIAVGTVIRYSCSGTFALIGEASLLCITKDKVDGTWDKPAPKCEYFNAYSSCPEPIVPGGYKIRGSTPYRHGDSVTFACKTNFSMNGNKSVWCQANNMWGPTRLPTCVSVFPLECPALPMIHNGHHTSENVGSIAPGLSVTYSCESGYLLVGEKIINCLSSGKWSAVPPTCEEARCKSLGRFPNGKVKEPPILRVGVTANFFCDEGYRLQGPPSSRCVIAGQGVAWTKMPVCGGGGSGGGGSEDCNELPPRRNTEILTGSWSDQTYPEGTQAIYKCRPGYRSLGNVIMVCRKGEWVALNPLRKCQKRPCGHPGDTPFGTFTLTGGNVFEYGVKAVYTCNEGYQLLGEINYRECDTDGWTNDIPICEVVKCLPVTAPENGKIVSSAMEPDREYHFGQAVRFVCNSGYKIEGDEEMHCSDDGFWSKEKPKCVEISCKSPDVINGSPISQKIIYKENERFQYKCNMGYEYSERGDAVCTESGWRPLPSCEIRVKTCSKSSIDIENGFISESQYTYALKEKAKYQCKLGYVTADGETSGSITCGKDGWSAQPTCIKSDSTGKCGPPPPIDNGDITSFPLSVYAPASSVEYQCQNLYQLEGNKRITCRNGQWSEPPKCLHPCVISREIMENYNIALRWTAKQKLYSRTGESVEFVCKRGYRLSSRSHTLRTTCWDGKLEYPTC

SEQ ID NO: 48 - protein, 724 aa, synthetic construct
MPMGSLQPLATLYLLGMLVASCLGISCGSPPPILNGRISYYSTPIAVGTVIRYSCSGTFALIGEASLLCITKDKVDGTWDKPAPKCEYFNAYSSCPEPIVPGGYKIRGSTPYRHGDSVTFACKTNFSMNGNKSVWCQANNMWGPTRLPTCVSVFPLECPALPMIHNGHHTSENVGSIAPGLSVTYSCESGYLLVGEKIINCLSSGKWSAVPPTCEEARCKSLGRFPNGKVKEPPILRVGVTANFFCDEGYRLQGPPSSRCVIAGQGVAWTKMPVCGGGGSGGGGSEDCNELPPRRNTEILTGSWSDQTYPEGTQAIYKCRPGYRSLGNVIMVCRKGEWVALNPLRKCQKRPCGHPGDTPFGTFTLTGGNVFEYGVKAVYTCNEGYQLLGEINYRECDTDGWTNDIPICEVVKCLPVTAPENGKIVSSAMEPDREYHFGQAVRFVCNSGYKIEGDEEMHCSDDGFWSKEKPKCVEISCKSPDVINGSPISQKIIYKENERFQYKCNMGYEYSERGDAVCTESGWRPLPSCEIRVKTCSKSSIDIENGFISESQYTYALKEKAKYQCKLGYVTADGETSGSITCGKDGWSAQPTCIKSDSTGKCGPPPPIDNGDITSFPLSVYAPASSVEYQCQNLYQLEGNKRITCRNGQWSEPPKCLHPCVISREIMENYNIALRWTAKQKLYSRTGESVEFVCKRGYRLSSRSHTLRTTCWDGKLEYPTCAKR

SEQ ID NO: 49 - protein, 689 aa, synthetic construct
CGSPPPILNGRISYYSTPIAVGTVIRYSCSGTFALIGEASLLCITKDKVDGTWDKPAPKCEYFNAYSSCPEPIVPGGYKIRGSTPYRHGDSVTFACKTNFSMNGNKSVWCQANNMWGPTRLPTCVSVFPLECPALPMIHNGHHTSENVGSIAPGLSVTYSCESGYLLVGEKIINCLSSGKWSAVPPTCEEARCKSLGRFPNGKVKEPPILRVGVTANFFCDEGYRLQGPPSSRCVIAGQGVAWTKMPVCGGGGSGGGGSEDCNELPPRRNTEILTGSWSDQTYPEGTQAIYKCRPGYRSLGNVIMVCRKGEWVALNPLRKCQKRPCGHPGDTPFGTFTLTGGNVFEYGVKAVYTCNEGYQLLGEINYRECDTDGWTNDIPICEVVKCLPVTAPENGKIVSSAMEPDREYHFGQAVRFVCNSGYKIEGDEEMHCSDDGFWSKEKPKCVEISCKSPDVINGSPISQKIIYKENERFQYKCNMGYEYSERGDAVCTESGWRPLPSCERDTSCVNPPTVQNAYIVSRQMSKYPSGERVRYQCRSPYEMFGDEEVMCLNGNWTEPPQCKDSTGKCGPPPPIDNGDITSFPLSVYAPASSVEYQCQNLYQLEGNKRITCRNGQWSEPPKCLHPCVISREIMENYNIALRWTAKQKLYSRTGESVEFVCKRGYRLSSRSHTLRTTCWDGKLEYPTC

SEQ ID NO: 50 - protein, 718 aa, synthetic construct
MPMGSLQPLATLYLLGMLVASCLGISCGSPPPILNGRISYYSTPIAVGTVIRYSCSGTFALIGEASLLCITKDKVDGTWDKPAPKCEYFNAYSSCPEPIVPGGYKIRGSTPYRHGDSVTFACKTNFSMNGNKSVWCQANNMWGPTRLPTCVSVFPLECPALPMIHNGHHTSENVGSIAPGLSVTYSCESGYLLVGEKIINCLSSGKWSAVPPTCEEARCKSLGRFPNGKVKEPPILRVGVTANFFCDEGYRLQGPPSSRCVIAGQGVAWTKMPVCGGGGSGGGGSEDCNELPPRRNTEILTGSWSDQTYPEGTQAIYKCRPGYRSLGNVIMVCRKGEWVALNPLRKCQKRPCGHPGDTPFGTFTLTGGNVFEYGVKAVYTCNEGYQLLGEINYRECDTDGWTNDIPICEVVKCLPVTAPENGKIVSSAMEPDREYHFGQAVRFVCNSGYKIEGDEEMHCSDDGFWSKEKPKCVEISCKSPDVINGSPISQKIIYKENERFQYKCNMGYEYSERGDAVCTESGWRPLPSCERDTSCVNPPTVQNAYIVSRQMSKYPSGERVRYQCRSPYEMFGDEEVMCLNGNWTEPPQCKDSTGKCGPPPPIDNGDITSFPLSVYAPASSVEYQCQNLYQLEGNKRITCRNGQWSEPPKCLHPCVISREIMENYNIALRWTAKQKLYSRTGESVEFVCKRGYRLSSRSHTLRTTCWDGKLEYPTCAKR

SEQ ID NO: 51 - protein, 758 aa, synthetic construct
CGSPPPILNGRISYYSTPIAVGTVIRYSCSGTFALIGEASLLCITKDKVDGTWDKPAPKCEYFNAYSSCPEPIVPGGYKIRGSTPYRHGDSVTFACKTNFSMNGNKSVWCQANNMWGPTRLPTCVSVFPLECPALPMIHNGHHTSENVGSIAPGLSVTYSCESGYLLVGEKIINCLSSGKWSAVPPTCEEARCKSLGRFPNGKVKEPPILRVGVTANFFCDEGYRLQGPPSSRCVIAGQGVAWTKMPVCGGGGSGGGGSEDCNELPPRRNTEILTGSWSDQTYPEGTQAIYKCRPGYRSLGNVIMVCRKGEWVALNPLRKCQKRPCGHPGDTPFGTFTLTGGNVFEYGVKAVYTCNEGYQLLGEINYRECDTDGWTNDIPICEVVKCLPVTAPENGKIVSSAMEPDREYHFGQAVRFVCNSGYKIEGDEEMHCSDDGFWSKEKPKCVEISCKSPDVINGSPISQKIIYKENERFQYKCNMGYEYSERGDAVCTESGWRPLPSCEGGGGSGGGGSEDCNELPPRRNTEILTGSWSDQTYPEGTQAIYKCRPGYRSLGNVIMVCRKGEWVALNPLRKCQKRPCGHPGDTPFGTFTLTGGNVFEYGVKAVYTCNEGYQLLGEINYRECDTDGWTNDIPICEVVKCLPVTAPENGKIVSSAMEPDREYHFGQAVRFVCNSGYKIEGDEEMHCSDDGFWSKEKPKCVEISCKSPDVINGSPISQKIIYKENERFQYKCNMGYEYSERGDAVCTESGWRPLPSC

SEQ ID NO: 52 - protein, 785 aa, synthetic construct
MPMGSLQPLATLYLLGMLVASCLGISCGSPPPILNGRISYYSTPIAVGTVIRYSCSGTFALIGEASLLCITKDKVDGTWDKPAPKCEYFNAYSSCPEPIVPGGYKIRGSTPYRHGDSVTFACKTNFSMNGNKSVWCQANNMWGPTRLPTCVSVFPLECPALPMIHNGHHTSENVGSIAPGLSVTYSCESGYLLVGEKIINCLSSGKWSAVPPTCEEARCKSLGRFPNGKVKEPPILRVGVTANFFCDEGYRLQGPPSSRCVIAGQGVAWTKMPVCGGGGSGGGGSEDCNELPPRRNTEILTGSWSDQTYPEGTQAIYKCRPGYRSLGNVIMVCRKGEWVALNPLRKCQKRPCGHPGDTPFGTFTLTGGNVFEYGVKAVYTCNEGYQLLGEINYRECDTDGWTNDIPICEVVKCLPVTAPENGKIVSSAMEPDREYHFGQAVRFVCNSGYKIEGDEEMHCSDDGFWSKEKPKCVEISCKSPDVINGSPISQKIIYKENERFQYKCNMGYEYSERGDAVCTESGWRPLPSCEGGGGSGGGGSEDCNELPPRRNTEILTGSWSDQTYPEGTQAIYKCRPGYRSLGNVIMVCRKGEWVALNPLRKCQKRPCGHPGDTPFGTFTLTGGNVFEYGVKAVYTCNEGYQLLGEINYRECDTDGWTNDIPICEVVKCLPVTAPENGKIVSSAMEPDREYHFGQAVRFVCNSGYKIEGDEEMHCSDDGFWSKEKPKCVEISCKSPDVINGSPISQKIIYKENERFQYKCNMGYEYSERGDAVCTESGWRPLPSCE

SEQ ID NO: 53 - protein, 631 aa, synthetic construct
CGSPPPILNGRISYYSTPIAVGTVIRYSCSGTFALIGEASLLCITKDKVDGTWDKPAPKCEYFNAYSSCPEPIVPGGYKIRGSTPYRHGDSVTFACKTNFSMNGNKSVWCQANNMWGPTRLPTCVSVFPLECPALPMIHNGHHTSENVGSIAPGLSVTYSCESGYLLVGEKIINCLSSGKWSAVPPTCEEARCKSLGRFPNGKVKEPPILRVGVTANFFCDEGYRLQGPPSSRCVIAGQGVAWTKMPVCGGGGSGGGGSEDCNELPPRRNTEILTGSWSDQTYPEGTQAIYKCRPGYRSLGNVIMVCRKGEWVALNPLRKCQKRPCGHPGDTPFGTFTLTGGNVFEYGVKAVYTCNEGYQLLGEINYRECDTDGWTNDIPICEVVKCLPVTAPENGKIVSSAMEPDREYHFGQAVRFVCNSGYKIEGDEEMHCSDDGFWSKEKPKCVEISCKSPDVINGSPISQKIIYKENERFQYKCNMGYEYSERGDAVCTESGWRPLPSCERDTSCVNPPTVQNAYIVSRQMSKYPSGERVRYQCRSPYEMFGDEEVMCLNGNWTEPPQCKDSTGKCVISREIMENYNIALRWTAKQKLYSRTGESVEFVCKRGYRLSSRSHTLRTTCWDGKLEYPTC

SEQ ID NO: 54 - protein, 660 aa, synthetic construct
MPMGSLQPLATLYLLGMLVASCLGISCGSPPPILNGRISYYSTPIAVGTVIRYSCSGTFALIGEASLLCITKDKVDGTWDKPAPKCEYFNAYSSCPEPIVPGGYKIRGSTPYRHGDSVTFACKTNFSMNGNKSVWCQANNMWGPTRLPTCVSVFPLECPALPMIHNGHHTSENVGSIAPGLSVTYSCESGYLLVGEKIINCLSSGKWSAVPPTCEEARCKSLGRFPNGKVKEPPILRVGVTANFFCDEGYRLQGPPSSRCVIAGQGVAWTKMPVCGGGGSGGGGSEDCNELPPRRNTEILTGSWSDQTYPEGTQAIYKCRPGYRSLGNVIMVCRKGEWVALNPLRKCQKRPCGHPGDTPFGTFTLTGGNVFEYGVKAVYTCNEGYQLLGEINYRECDTDGWTNDIPICEVVKCLPVTAPENGKIVSSAMEPDREYHFGQAVRFVCNSGYKIEGDEEMHCSDDGFWSKEKPKCVEISCKSPDVINGSPISQKIIYKENERFQYKCNMGYEYSERGDAVCTESGWRPLPSCERDTSCVNPPTVQNAYIVSRQMSKYPSGERVRYQCRSPYEMFGDEEVMCLNGNWTEPPQCKDSTGKCVISREIMENYNIALRWTAKQKLYSRTGESVEFVCKRGYRLSSRSHTLRTTCWDGKLEYPTCAKR

SEQ ID NO: 55 - protein, 826 aa, synthetic construct
CGSPPPILNGRISYYSTPIAVGTVIRYSCSGTFALIGEASLLCITKDKVDGTWDKPAPKCEYFNAYSSCPEPIVPGGYKIRGSTPYRHGDSVTFACKTNFSMNGNKSVWCQANNMWGPTRLPTCVSVFPLECPALPMIHNGHHTSENVGSIAPGLSVTYSCESGYLLVGEKIINCLSSGKWSAVPPTCEEARCKSLGRFPNGKVKEPPILRVGVTANFFCDEGYRLQGPPSSRCVIAGQGVAWTKMPVCGGGGSGGGGSEDCNELPPRRNTEILTGSWSDQTYPEGTQAIYKCRPGYRSLGNVIMVCRKGEWVALNPLRKCQKRPCGHPGDTPFGTFTLTGGNVFEYGVKAVYTCNEGYQLLGEINYRECDTDGWTNDIPICEVVKCLPVTAPENGKIVSSAMEPDREYHFGQAVRFVCNSGYKIEGDEEMHCSDDGFWSKEKPKCVEISCKSPDVINGSPISQKIIYKENERFQYKCNMGYEYSERGDAVCTESGWRPLPSCEGGGGSGGGGSEDCNELPPRRNTEILTGSWSDQTYPEGTQAIYKCRPGYRSLGNVIMVCRKGEWVALNPLRKCQKRPCGHPGDTPFGTFTLTGGNVFEYGVKAVYTCNEGYQLLGEINYRECDTDGWTNDIPICEVVKCLPVTAPENGKIVSSAMEPDREYHFGQAVRFVCNSGYKIEGDEEMHCSDDGFWSKEKPKCVEISCKSPDVINGSPISQKIIYKENERFQYKCNMGYEYSERGDAVCTESGWRPLPSCEGGGGSGGGGSLRKCYFPYLENGYNQNHGRKFVQGKSIDVACHPGYALPKAQTTVTCMENGWSPTPRC

SEQ ID NO: 56 - protein, 857 aa, synthetic construct
MPMGSLQPLATLYLLGMLVASCLGISCGSPPPILNGRISYYSTPIAVGTVIRYSCSGTFALIGEASLLCITKDKVDGTWDKPAPKCEYFNAYSSCPEPIVPGGYKIRGSTPYRHGDSVTFACKTNFSMNGNKSVWCQANNMWGPTRLPTCVSVFPLECPALPMIHNGHHTSENVGSIAPGLSVTYSCESGYLLVGEKIINCLSSGKWSAVPPTCEEARCKSLGRFPNGKVKEPPILRVGVTANFFCDEGYRLQGPPSSRCVIAGQGVAWTKMPVCGGGGSGGGGSEDCNELPPRRNTEILTGSWSDQTYPEGTQAIYKCRPGYRSLGNVIMVCRKGEWVALNPLRKCQKRPCGHPGDTPFGTFTLTGGNVFEYGVKAVYTCNEGYQLLGEINYRECDTDGWTNDIPICEVVKCLPVTAPENGKIVSSAMEPDREYHFGQAVRFVCNSGYKIEGDEEMHCSDDGFWSKEKPKCVEISCKSPDVINGSPISQKIIYKENERFQYKCNMGYEYSERGDAVCTESGWRPLPSCEGGGGSGGGGSEDCNELPPRRNTEILTGSWSDQTYPEGTQAIYKCRPGYRSLGNVIMVCRKGEWVALNPLRKCQKRPCGHPGDTPFGTFTLTGGNVFEYGVKAVYTCNEGYQLLGEINYRECDTDGWTNDIPICEVVKCLPVTAPENGKIVSSAMEPDREYHFGQAVRFVCNSGYKIEGDEEMHCSDDGFWSKEKPKCVEISCKSPDVINGSPISQKIIYKENERFQYKCNMGYEYSERGDAVCTESGWRPLPSCEGGGGSGGGGSLRKCYFPYLENGYNQNHGRKFVQGKSIDVACHPGYALPKAQTTVTCMENGWSPTPRCIRVKT

SEQ ID NO: 57 - DNA, 165 bp, synthetic construct
  source 1..165: mol_type = other DNA
tgcgtgaaccctccaacagtccaaaatgcctatatagtctctaggcagatgagtaaatacccaagtggagagagagtgagataccagtgccggtctccttacgagatgttcggcgacgaggaagtgatgtgcctgaacggcaattggacagagccaccacaatgt

SEQ ID NO: 58 - DNA, 186 bp, synthetic construct
  source 1..186: mol_type = other DNA
tgtgtgatcagtcgggagatcatggagaactacaacattgccctgaggtggactgctaagcagaagctctatagccgaacaggcgagtcagtggagtttgtgtgtaaacggggatacaggctgtccagtaggagccacaccctgcgcactacttgctgggatgggaagctggaatatccaacttgc

SEQ ID NO: 59 - DNA, 1893 bp, synthetic construct
  source 1..1893: mol_type = other DNA
tgcggctctcctccacccattctcaatggaaggatctcctactacagcacccccatagctgtcggcaccgttatccgatacagttgttccggtactttccggcttatcggcgaaaagtctttgctgtgcattaccaaggataaagtggacgggacttgggacaaacccgcacctaagtgcgagtattttaacaaatatagcagctgccctgagcctatagtacccggggggtataaaatccggggctctactccctatcgtcatggcgattctgtgaccttcgcatgtaaaactaatttttcaatgaatggcaacaagtctgtatggtgtcaagcaaataacatgtggggacctacccgcctgccaacctgtgtgtcagtgtttcccctggaatgtccagccctccctatgatccacaacggacatcacaccagcgaaaacgttggctccatcgcaccagggctctctgtgacttactcttgcgagtccgggtacctgctcgtgggtgaaaagatcatcaactgcctcagtagtggtaaatggtccgccgtgcctcccacatgtgaagaggcccggtgcaagagcctgggccggttccccaacggaaaagtgaaggaacctcctatcttgagggttggtgtgaccgctaactttttctgcgacgaggggtacaggctccaagggcctccctctagtcggtgcgtaatcgccggtcaaggagtcgcatggactaagatgcctgtgtgtggcggaggtgggtcgggtggcggcggatctgaggactgcaacgaactgcctcctagaagaaacaccgaaatcctcacaggctcctggtcagatcagacctaccctgagggtacacaggccatctataaatgccgcccgggttaccgctccttgggcaatgttattatggtctgccggaaaggggaatgggtggccttgaaccccctcagaaagtgccaaaaaagaccctgcggacatccaggagacacacctttcgggacatttaccttgaccggtggtaacgtgttcgagtacggagtgaaggcagtctatacttgcaatgagggctaccagctcctgggggaaataaattatcgcgaatgtgatacagacggctggacgaacgacattcctatctgtgaggtggtcaaatgtctgcccgtcactgctcctgaaaacggcaagatagtgagttctgcaatggagccggatagggagtatcattttggtcaggccgtgcgctttgtgtgcaatagtgggtataaaatcgagggggatgaagaaatgcactgtagcgacgatggattctggtctaaagagaaacctaagtgtgtggagattagttgcaagagtccagacgtgattaacggtagccccatttcccaaaagataatatacaaggaaaacgaaagattccagtataaatgcaacatgggctacgagtatagcgagcggggcgatgccgtgtgtactgaaagcggctggcgccccctgccttcctgcgagcgggatacaagctgcgtgaaccctccaacagtccaaaatgcctatatagtctctaggcagatgagtaaatacccaagtggagagagagtgagataccagtgccggtctccttacgagatgttcggcgacgaggaagtgatgtgcctgaacggcaattggacagagccaccacaatgtaaggatagtacaggcaaatgtgtgatcagtcgggagatcatggagaactacaacattgccctgaggtggactgctaagcagaagctctatagccgaacaggcgagtcagtggagtttgtgtgtaaacggggatacaggctgtccagtaggagccacaccctgcgcactacttgctgggatgggaagctggaatatccaacttgc

SEQ ID NO: 60 - DNA, 1980 bp, synthetic construct
  source 1..1980: mol_type = other DNA
atgccaatggggtccctacaacccctggcaacactatatctgctaggtatgctcgtggcctcctgtttaggaatttcatgcggctctcctccacccattctcaatggaaggatctcctactacagcacccccatagctgtcggcaccgttatccgatacagttgttccggtactttccggcttatcggcgaaaagtctttgctgtgcattaccaaggataaagtggacgggacttgggacaaacccgcacctaagtgcgagtattttaacaaatatagcagctgccctgagcctatagtacccggggggtataaaatccggggctctactccctatcgtcatggcgattctgtgaccttcgcatgtaaaactaatttttcaatgaatggcaacaagtctgtatggtgtcaagcaaataacatgtggggacctacccgcctgccaacctgtgtgtcagtgtttcccctggaatgtccagccctccctatgatccacaacggacatcacaccagcgaaaacgttggctccatcgcaccagggctctctgtgacttactcttgcgagtccgggtacctgctcgtgggtgaaaagatcatcaactgcctcagtagtggtaaatggtccgccgtgcctcccacatgtgaagaggcccggtgcaagagcctgggccggttccccaacggaaaagtgaaggaacctcctatcttgagggttggtgtgaccgctaactttttctgcgacgaggggtacaggctccaagggcctccctctagtcggtgcgtaatcgccggtcaaggagtcgcatggactaagatgcctgtgtgtggcggaggtgggtcgggtggcggcggatctgaggactgcaacgaactgcctcctagaagaaacaccgaaatcctcacaggctcctggtcagatcagacctaccctgagggtacacaggccatctataaatgccgcccgggttaccgctccttgggcaatgttattatggtctgccggaaaggggaatgggtggccttgaaccccctcagaaagtgccaaaaaagaccctgcggacatccaggagacacacctttcgggacatttaccttgaccggtggtaacgtgttcgagtacggagtgaaggcagtctatacttgcaatgagggctaccagctcctgggggaaataaattatcgcgaatgtgatacagacggctggacgaacgacattcctatctgtgaggtggtcaaatgtctgcccgtcactgctcctgaaaacggcaagatagtgagttctgcaatggagccggatagggagtatcattttggtcaggccgtgcgctttgtgtgcaatagtgggtataaaatcgagggggatgaagaaatgcactgtagcgacgatggattctggtctaaagagaaacctaagtgtgtggagattagttgcaagagtccagacgtgattaacggtagccccatttcccaaaagataatatacaaggaaaacgaaagattccagtataaatgcaacatgggctacgagtatagcgagcggggcgatgccgtgtgtactgaaagcggctggcgccccctgccttcctgcgagcgggatacaagctgcgtgaaccctccaacagtccaaaatgcctatatagtctctaggcagatgagtaaatacccaagtggagagagagtgagataccagtgccggtctccttacgagatgttcggcgacgaggaagtgatgtgcctgaacggcaattggacagagccaccacaatgtaaggatagtacaggcaaatgtgtgatcagtcgggagatcatggagaactacaacattgccctgaggtggactgctaagcagaagctctatagccgaacaggcgagtcagtggagtttgtgtgtaaacggggatacaggctgtccagtaggagccacaccctgcgcactacttgctgggatgggaagctggaatatccaacttgcgccaagagg

SEQ ID NO: 61 - DNA, 162 bp, synthetic construct
  source 1..162: mol_type = other DNA
tgttacttcccctacctggagaacggctacaatcagaaccacggcagaaagttcgtgcaaggcaagagcatcgacgtggcctgccaccccggctacgccctgcccaaggctcagaccaccgtgacctgcatggagaatggctggagccccacccctagatgc

SEQ ID NO: 62 - DNA, 2478 bp, synthetic construct
  source 1..2478: mol_type = other DNA
tgcggcagcccccctcccatcctgaacggcagaatcagctactacagcacccccatcgccgtgggcaccgtgatcagatacagctgcagcggcaccttcagactgatcggcgagaagagcctgctgtgcatcaccaaggacaaggtggacggcacctgggacaagcccgcccccaagtgcgagtacttcaacaagtacagcagctgccccgagcccatcgtgcctggcggctacaagatcagaggcagcaccccctacagacacggcgacagcgtgaccttcgcctgcaagaccaacttcagcatgaacggcaacaagagcgtgtggtgccaagccaacaacatgtggggccccacaagactgcccacctgcgtgagcgtgttccccctggagtgccccgccctgcccatgatccacaacggccaccacacaagcgagaacgtgggcagcatcgcccccggcctgagcgtgacctacagctgcgagagcggctacctgctggtgggcgagaagatcatcaactgcctgagcagcggcaagtggagcgccgtgccccccacctgcgaggaggctagatgcaagagcctgggcagattccccaacggcaaggtgaaggagcctcctatcctgagagtgggcgtgaccgccaacttcttctgcgacgagggctacagactgcaaggcccccctagcagcagatgtgtgatcgctggccaaggcgtggcctggaccaaaatgcccgtctgcgggggggggggcagcgggggcgggggcagcgaggattgcaacgagctgccccctagacggaacacagagatcctgaccggcagctggagcgatcaaacatatcccgagggcacccaagccatctacaaatgcagacctggctacagaagcctgggcaatgtgatcatggtctgccggaaaggggagtgggtcgctctgaaccccctgcggaagtgtcagaagagaccttgcggccaccccggcgacacacccttcgggaccttcacactgaccggcggcaacgtgtttgagtacggcgtcaaggccgtgtacacctgtaacgaggggtatcagctgctgggcgagatcaactacagagagtgcgataccgacggctggaccaatgacatccccatctgcgaggtggtgaagtgtctgcccgtgaccgcccccgaaaacggcaagatcgtgagcagcgccatggagcccgaccgggagtaccattttgggcaagctgtgagattcgtctgcaatagcggctacaagatcgaaggcgacgaggagatgcactgtagcgacgacggcttctggtccaaagagaaacccaaatgcgtggagatctcctgcaaaagccccgatgtgatcaacggcagccccatctcccaaaaaattatctacaaggaaaacgaacggtttcagtacaaatgcaacatgggctacgaatactccgagcggggggatgccgtgtgcaccgagagcggctggcggcctctgcctagctgtgaagggggcggcgggagcggcgggggcggcagcgaggactgcaatgaactgcctcctagacggaacaccgaaatcctgaccgggagctggagcgaccaaacataccccgaggggacacaagccatctacaagtgcagacctgggtatagatccctcgggaacgtgatcatggtctgtcggaagggcgagtgggtcgctctgaaccctctcagaaagtgtcagaaacggccctgcgggcaccccggcgatacccccttcggcacattcaccctgaccggggggaacgtgttcgagtacggcgtgaaggccgtctacacctgcaacgagggctaccaactcctgggcgaaatcaattacagagaatgcgacacagatggctggaccaacgacatccctatctgcgaggtcgtgaaatgtctccccgtgacagcccctgagaacggcaagattgtcagcagcgctatggaacctgatagagagtaccatttcggccaagccgtcagatttgtgtgcaattccggctacaaaattgagggggacgaagagatgcactgctccgacgatggcttctggagcaaggaaaaacccaagtgcgtggagattagctgcaagagccccgacgtgatcaacgggagccccatctcccaaaaaatcatctacaaggagaacgagagatttcagtataagtgcaacatgggctatgagtacagcgagcggggggacgccgtgtgtaccgaatccgggtggagacccctgcctagctgcgagggcgggggcgggagcggcgggggcggctccctgagaaagtgttacttcccctacctggagaacggctacaatcagaaccacggcagaaagttcgtgcaaggcaagagcatcgacgtggcctgccaccccggctacgccctgcccaaggctcagaccaccgtgacctgcatggagaatggctggagccccacccctagatgc

SEQ ID NO: 63 - DNA, 2574 bp, synthetic construct
  source 1..2574: mol_type = other DNA
atgcccatgggcagcctgcagcccctggccaccctgtacctgctgggcatgctggtggctagctgcctgggcatcagctgcggcagcccccctcccatcctgaacggcagaatcagctactacagcacccccatcgccgtgggcaccgtgatcagatacagctgcagcggcaccttcagactgatcggcgagaagagcctgctgtgcatcaccaaggacaaggtggacggcacctgggacaagcccgcccccaagtgcgagtacttcaacaagtacagcagctgccccgagcccatcgtgcctggcggctacaagatcagaggcagcaccccctacagacacggcgacagcgtgaccttcgcctgcaagaccaacttcagcatgaacggcaacaagagcgtgtggtgccaagccaacaacatgtggggccccacaagactgcccacctgcgtgagcgtgttccccctggagtgccccgccctgcccatgatccacaacggccaccacacaagcgagaacgtgggcagcatcgcccccggcctgagcgtgacctacagctgcgagagcggctacctgctggtgggcgagaagatcatcaactgcctgagcagcggcaagtggagcgccgtgccccccacctgcgaggaggctagatgcaagagcctgggcagattccccaacggcaaggtgaaggagcctcctatcctgagagtgggcgtgaccgccaacttcttctgcgacgagggctacagactgcaaggcccccctagcagcagatgtgtgatcgctggccaaggcgtggcctggaccaaaatgcccgtctgcgggggggggggcagcgggggcgggggcagcgaggattgcaacgagctgccccctagacggaacacagagatcctgaccggcagctggagcgatcaaacatatcccgagggcacccaagccatctacaaatgcagacctggctacagaagcctgggcaatgtgatcatggtctgccggaaaggggagtgggtcgctctgaaccccctgcggaagtgtcagaagagaccttgcggccaccccggcgacacacccttcgggaccttcacactgaccggcggcaacgtgtttgagtacggcgtcaaggccgtgtacacctgtaacgaggggtatcagctgctgggcgagatcaactacagagagtgcgataccgacggctggaccaatgacatccccatctgcgaggtggtgaagtgtctgcccgtgaccgcccccgaaaacggcaagatcgtgagcagcgccatggagcccgaccgggagtaccattttgggcaagctgtgagattcgtctgcaatagcggctacaagatcgaaggcgacgaggagatgcactgtagcgacgacggcttctggtccaaagagaaacccaaatgcgtggagatctcctgcaaaagccccgatgtgatcaacggcagccccatctcccaaaaaattatctacaaggaaaacgaacggtttcagtacaaatgcaacatgggctacgaatactccgagcggggggatgccgtgtgcaccgagagcggctggcggcctctgcctagctgtgaagggggcggcgggagcggcgggggcggcagcgaggactgcaatgaactgcctcctagacggaacaccgaaatcctgaccgggagctggagcgaccaaacataccccgaggggacacaagccatctacaagtgcagacctgggtatagatccctcgggaacgtgatcatggtctgtcggaagggcgagtgggtcgctctgaaccctctcagaaagtgtcagaaacggccctgcgggcaccccggcgatacccccttcggcacattcaccctgaccggggggaacgtgttcgagtacggcgtgaaggccgtctacacctgcaacgagggctaccaactcctgggcgaaatcaattacagagaatgcgacacagatggctggaccaacgacatccctatctgcgaggtcgtgaaatgtctccccgtgacagcccctgagaacggcaagattgtcagcagcgctatggaacctgatagagagtaccatttcggccaagccgtcagatttgtgtgcaattccggctacaaaattgagggggacgaagagatgcactgctccgacgatggcttctggagcaaggaaaaacccaagtgcgtggagattagctgcaagagccccgacgtgatcaacgggagccccatctcccaaaaaatcatctacaaggagaacgagagatttcagtataagtgcaacatgggctatgagtacagcgagcggggggacgccgtgtgtaccgaatccgggtggagacccctgcctagctgcgagggcgggggcgggagcggcgggggcggctccctgagaaagtgttacttcccctacctggagaacggctacaatcagaaccacggcagaaagttcgtgcaaggcaagagcatcgacgtggcctgccaccccggctacgccctgcccaaggctcagaccaccgtgacctgcatggagaatggctggagccccacccctagatgcatcagagtgaagacctac

SEQ ID NO: 64 - DNA, 747 bp, synthetic construct
  source 1..747: mol_type = other DNA
tgtggcagccctcctcctattctgaatggcaggatcagctactacagcacccctattgccgtgggcaccgtgatcagatacagctgctctggcacattcgccctgatcggcgaagccagcctgctgtgcatcaccaaggataaggtggacggcacctgggacaagcccgctcctaagtgcgaatatttcaacgcctacagcagctgccctgagcctattgtgcctggcggctacaagatcagaggcagcaccccatacagacacggcgacagcgtgacctttgcctgcaagaccaacttcagcatgaacggcaacaagagcgtgtggtgccaggccaacaatatgtggggccctaccagactgcccacctgtgtgtctgtgttccctctggaatgccccgctctgcccatgatccacaatggccaccacaccagcgagaacgtgggatctattgcccctggcctgtccgtgacctacagctgtgaaagcggctatctgctcgtgggcgagaagatcatcaactgcctgagcagcggcaagtggagcgctgttcctcctacatgcgaagaggccagatgcaagagcctgggcagattccccaacggcaaagtgaaagagcctcctatcctgagagtgggcgtgaccgccaacttcttctgcgacgagggctacagactgcagggccctcctagcagcagatgtgtgattgctggacagggcgtcgcctggaccaagatgcctgtttgt

SEQ ID NO: 65 - DNA, 2085 bp, synthetic construct
  source 1..2085: mol_type = other DNA
tgtggcagccctcctcctattctgaatggcaggatcagctactacagcacccctattgccgtgggcaccgtgatcagatacagctgctctggcacattcgccctgatcggcgaagccagcctgctgtgcatcaccaaggataaggtggacggcacctgggacaagcccgctcctaagtgcgaatatttcaacgcctacagcagctgccctgagcctattgtgcctggcggctacaagatcagaggcagcaccccatacagacacggcgacagcgtgacctttgcctgcaagaccaacttcagcatgaacggcaacaagagcgtgtggtgccaggccaacaatatgtggggccctaccagactgcccacctgtgtgtctgtgttccctctggaatgccccgctctgcccatgatccacaatggccaccacaccagcgagaacgtgggatctattgcccctggcctgtccgtgacctacagctgtgaaagcggctatctgctcgtgggcgagaagatcatcaactgcctgagcagcggcaagtggagcgctgttcctcctacatgcgaagaggccagatgcaagagcctgggcagattccccaacggcaaagtgaaagagcctcctatcctgagagtgggcgtgaccgccaacttcttctgcgacgagggctacagactgcagggccctcctagcagcagatgtgtgattgctggacagggcgtcgcctggaccaagatgcctgtttgtggcggaggtgggtcgggtggcggcggatctgaggactgcaacgaactgcctcctagaagaaacaccgaaatcctcacaggctcctggtcagatcagacctaccctgagggtacacaggccatctataaatgccgcccgggttaccgctccttgggcaatgttattatggtctgccggaaaggggaatgggtggccttgaaccccctcagaaagtgccaaaaaagaccctgcggacatccaggagacacacctttcgggacatttaccttgaccggtggtaacgtgttcgagtacggagtgaaggcagtctatacttgcaatgagggctaccagctcctgggggaaataaattatcgcgaatgtgatacagacggctggacgaacgacattcctatctgtgaggtggtcaaatgtctgcccgtcactgctcctgaaaacggcaagatagtgagttctgcaatggagccggatagggagtatcattttggtcaggccgtgcgctttgtgtgcaatagtgggtataaaatcgagggggatgaagaaatgcactgtagcgacgatggattctggtctaaagagaaacctaagtgtgtggagattagttgcaagagtccagacgtgattaacggtagccccatttcccaaaagataatatacaaggaaaacgaaagattccagtataaatgcaacatgggctacgagtatagcgagcggggcgatgccgtgtgtactgaaagcggctggcgccccctgccttcctgcgagattagggtgaagacctgttccaaaagcagcatcgacatcgaaaacggctttatatccgagagccagtatacgtatgcgctgaaggaaaaggccaagtatcagtgcaagctcggttatgtcacagctgatggcgagacctccgggtctatcacatgcggcaaagacggctggtccgctcagcctacctgcattaagagcgatagtacaggcaaatgtgggccacctcccccaattgataatggtgatataacctccttccctcttagtgtttacgccccagcatccagcgtggagtatcaatgccaaaatctgtaccaactggaggggaacaaacggataacctgccgcaacggccaatggtccgagccacctaagtgcctgcatccatgtgtgatcagtcgggagatcatggagaactacaacattgccctgaggtggactgctaagcagaagctctatagccgaacaggcgagtcagtggagtttgtgtgtaaacggggatacaggctgtccagtaggagccacaccctgcgcactacttgctgggatgggaagctggaatatccaacttgc

SEQ ID NO: 66 - DNA, 2172 bp, synthetic construct
  source 1..2172: mol_type = other DNA
atgccaatggggtccctacaacccctggcaacactatatctgctaggtatgctcgtggcctcctgtttaggaatcagctgtggcagccctcctcctattctgaatggcaggatcagctactacagcacccctattgccgtgggcaccgtgatcagatacagctgctctggcacattcgccctgatcggcgaagccagcctgctgtgcatcaccaaggataaggtggacggcacctgggacaagcccgctcctaagtgcgaatatttcaacgcctacagcagctgccctgagcctattgtgcctggcggctacaagatcagaggcagcaccccatacagacacggcgacagcgtgacctttgcctgcaagaccaacttcagcatgaacggcaacaagagcgtgtggtgccaggccaacaatatgtggggccctaccagactgcccacctgtgtgtctgtgttccctctggaatgccccgctctgcccatgatccacaatggccaccacaccagcgagaacgtgggatctattgcccctggcctgtccgtgacctacagctgtgaaagcggctatctgctcgtgggcgagaagatcatcaactgcctgagcagcggcaagtggagcgctgttcctcctacatgcgaagaggccagatgcaagagcctgggcagattccccaacggcaaagtgaaagagcctcctatcctgagagtgggcgtgaccgccaacttcttctgcgacgagggctacagactgcagggccctcctagcagcagatgtgtgattgctggacagggcgtcgcctggaccaagatgcctgtttgtggcggaggtgggtcgggtggcggcggatctgaggactgcaacgaactgcctcctagaagaaacaccgaaatcctcacaggctcctggtcagatcagacctaccctgagggtacacaggccatctataaatgccgcccgggttaccgctccttgggcaatgttattatggtctgccggaaaggggaatgggtggccttgaaccccctcagaaagtgccaaaaaagaccctgcggacatccaggagacacacctttcgggacatttaccttgaccggtggtaacgtgttcgagtacggagtgaaggcagtctatacttgcaatgagggctaccagctcctgggggaaataaattatcgcgaatgtgatacagacggctggacgaacgacattcctatctgtgaggtggtcaaatgtctgcccgtcactgctcctgaaaacggcaagatagtgagttctgcaatggagccggatagggagtatcattttggtcaggccgtgcgctttgtgtgcaatagtgggtataaaatcgagggggatgaagaaatgcactgtagcgacgatggattctggtctaaagagaaacctaagtgtgtggagattagttgcaagagtccagacgtgattaacggtagccccatttcccaaaagataatatacaaggaaaacgaaagattccagtataaatgcaacatgggctacgagtatagcgagcggggcgatgccgtgtgtactgaaagcggctggcgccccctgccttcctgcgagattagggtgaagacctgttccaaaagcagcatcgacatcgaaaacggctttatatccgagagccagtatacgtatgcgctgaaggaaaaggccaagtatcagtgcaagctcggttatgtcacagctgatggcgagacctccgggtctatcacatgcggcaaagacggctggtccgctcagcctacctgcattaagagcgatagtacaggcaaatgtgggccacctcccccaattgataatggtgatataacctccttccctcttagtgtttacgccccagcatccagcgtggagtatcaatgccaaaatctgtaccaactggaggggaacaaacggataacctgccgcaacggccaatggtccgagccacctaagtgcctgcatccatgtgtgatcagtcgggagatcatggagaactacaacattgccctgaggtggactgctaagcagaagctctatagccgaacaggcgagtcagtggagtttgtgtgtaaacggggatacaggctgtccagtaggagccacaccctgcgcactacttgctgggatgggaagctggaatatccaacttgcgccaagagg

SEQ ID NO: 67 - DNA, 2067 bp, synthetic construct
  source 1..2067: mol_type = other DNA
tgtggcagccctcctcctattctgaatggcaggatcagctactacagcacccctattgccgtgggcaccgtgatcagatacagctgctctggcacattcgccctgatcggcgaagccagcctgctgtgcatcaccaaggataaggtggacggcacctgggacaagcccgctcctaagtgcgaatatttcaacgcctacagcagctgccctgagcctattgtgcctggcggctacaagatcagaggcagcaccccatacagacacggcgacagcgtgacctttgcctgcaagaccaacttcagcatgaacggcaacaagagcgtgtggtgccaggccaacaatatgtggggccctaccagactgcccacctgtgtgtctgtgttccctctggaatgccccgctctgcccatgatccacaatggccaccacaccagcgagaacgtgggatctattgcccctggcctgtccgtgacctacagctgtgaaagcggctatctgctcgtgggcgagaagatcatcaactgcctgagcagcggcaagtggagcgctgttcctcctacatgcgaagaggccagatgcaagagcctgggcagattccccaacggcaaagtgaaagagcctcctatcctgagagtgggcgtgaccgccaacttcttctgcgacgagggctacagactgcagggccctcctagcagcagatgtgtgattgctggacagggcgtcgcctggaccaagatgcctgtttgtggcggaggtgggtcgggtggcggcggatctgaggactgcaacgaactgcctcctagaagaaacaccgaaatcctcacaggctcctggtcagatcagacctaccctgagggtacacaggccatctataaatgccgcccgggttaccgctccttgggcaatgttattatggtctgccggaaaggggaatgggtggccttgaaccccctcagaaagtgccaaaaaagaccctgcggacatccaggagacacacctttcgggacatttaccttgaccggtggtaacgtgttcgagtacggagtgaaggcagtctatacttgcaatgagggctaccagctcctgggggaaataaattatcgcgaatgtgatacagacggctggacgaacgacattcctatctgtgaggtggtcaaatgtctgcccgtcactgctcctgaaaacggcaagatagtgagttctgcaatggagccggatagggagtatcattttggtcaggccgtgcgctttgtgtgcaatagtgggtataaaatcgagggggatgaagaaatgcactgtagcgacgatggattctggtctaaagagaaacctaagtgtgtggagattagttgcaagagtccagacgtgattaacggtagccccatttcccaaaagataatatacaaggaaaacgaaagattccagtataaatgcaacatgggctacgagtatagcgagcggggcgatgccgtgtgtactgaaagcggctggcgccccctgccttcctgcgagcgggatacaagctgcgtgaaccctccaacagtccaaaatgcctatatagtctctaggcagatgagtaaatacccaagtggagagagagtgagataccagtgccggtctccttacgagatgttcggcgacgaggaagtgatgtgcctgaacggcaattggacagagccaccacaatgtaaggatagtacaggcaaatgtgggccacctcccccaattgataatggtgatataacctccttccctcttagtgtttacgccccagcatccagcgtggagtatcaatgccaaaatctgtaccaactggaggggaacaaacggataacctgccgcaacggccaatggtccgagccacctaagtgcctgcatccatgtgtgatcagtcgggagatcatggagaactacaacattgccctgaggtggactgctaagcagaagctctatagccgaacaggcgagtcagtggagtttgtgtgtaaacggggatacaggctgtccagtaggagccacaccctgcgcactacttgctgggatgggaagctggaatatccaacttgc

SEQ ID NO: 68 - DNA, 2154 bp, synthetic construct
  source 1..2154: mol_type = other DNA
atgccaatggggtccctacaacccctggcaacactatatctgctaggtatgctcgtggcctcctgtttaggaatcagctgtggcagccctcctcctattctgaatggcaggatcagctactacagcacccctattgccgtgggcaccgtgatcagatacagctgctctggcacattcgccctgatcggcgaagccagcctgctgtgcatcaccaaggataaggtggacggcacctgggacaagcccgctcctaagtgcgaatatttcaacgcctacagcagctgccctgagcctattgtgcctggcggctacaagatcagaggcagcaccccatacagacacggcgacagcgtgacctttgcctgcaagaccaacttcagcatgaacggcaacaagagcgtgtggtgccaggccaacaatatgtggggccctaccagactgcccacctgtgtgtctgtgttccctctggaatgccccgctctgcccatgatccacaatggccaccacaccagcgagaacgtgggatctattgcccctggcctgtccgtgacctacagctgtgaaagcggctatctgctcgtgggcgagaagatcatcaactgcctgagcagcggcaagtggagcgctgttcctcctacatgcgaagaggccagatgcaagagcctgggcagattccccaacggcaaagtgaaagagcctcctatcctgagagtgggcgtgaccgccaacttcttctgcgacgagggctacagactgcagggccctcctagcagcagatgtgtgattgctggacagggcgtcgcctggaccaagatgcctgtttgtggcggaggtgggtcgggtggcggcggatctgaggactgcaacgaactgcctcctagaagaaacaccgaaatcctcacaggctcctggtcagatcagacctaccctgagggtacacaggccatctataaatgccgcccgggttaccgctccttgggcaatgttattatggtctgccggaaaggggaatgggtggccttgaaccccctcagaaagtgccaaaaaagaccctgcggacatccaggagacacacctttcgggacatttaccttgaccggtggtaacgtgttcgagtacggagtgaaggcagtctatacttgcaatgagggctaccagctcctgggggaaataaattatcgcgaatgtgatacagacggctggacgaacgacattcctatctgtgaggtggtcaaatgtctgcccgtcactgctcctgaaaacggcaagatagtgagttctgcaatggagccggatagggagtatcattttggtcaggccgtgcgctttgtgtgcaatagtgggtataaaatcgagggggatgaagaaatgcactgtagcgacgatggattctggtctaaagagaaacctaagtgtgtggagattagttgcaagagtccagacgtgattaacggtagccccatttcccaaaagataatatacaaggaaaacgaaagattccagtataaatgcaacatgggctacgagtatagcgagcggggcgatgccgtgtgtactgaaagcggctggcgccccctgccttcctgcgagcgggatacaagctgcgtgaaccctccaacagtccaaaatgcctatatagtctctaggcagatgagtaaatacccaagtggagagagagtgagataccagtgccggtctccttacgagatgttcggcgacgaggaagtgatgtgcctgaacggcaattggacagagccaccacaatgtaaggatagtacaggcaaatgtgggccacctcccccaattgataatggtgatataacctccttccctcttagtgtttacgccccagcatccagcgtggagtatcaatgccaaaatctgtaccaactggaggggaacaaacggataacctgccgcaacggccaatggtccgagccacctaagtgcctgcatccatgtgtgatcagtcgggagatcatggagaactacaacattgccctgaggtggactgctaagcagaagctctatagccgaacaggcgagtcagtggagtttgtgtgtaaacggggatacaggctgtccagtaggagccacaccctgcgcactacttgctgggatgggaagctggaatatccaacttgcgccaagagg

SEQ ID NO: 69 - DNA, 747 bp, synthetic construct
  source 1..747: mol_type = other DNA
tgcggcagcccccctcccatcctgaacggcagaatcagctactacagcacccccatcgccgtgggcaccgtgatcagatacagctgcagcggcaccttcgccctgatcggcgaggctagcctgctgtgcatcaccaaggacaaggtggacggcacctgggacaagcccgcccccaagtgcgagtacttcaacgcctacagcagctgccccgagcccatcgtgcctggcggctacaagatcagaggcagcaccccctacagacacggcgacagcgtgaccttcgcctgcaagaccaacttcagcatgaacggcaacaagagcgtgtggtgccaagccaacaacatgtggggccccacaagactgcccacctgcgtgagcgtgttccccctggagtgccccgccctgcccatgatccacaacggccaccacacaagcgagaacgtgggcagcatcgcccccggcctgagcgtgacctacagctgcgagagcggctacctgctggtgggcgagaagatcatcaactgcctgagcagcggcaagtggagcgccgtgccccccacctgcgaggaggctagatgcaagagcctgggcagattccccaacggcaaggtgaaggagcctcctatcctgagagtgggcgtgaccgccaacttcttctgcgacgagggctacagactgcaaggcccccctagcagcagatgtgtgatcgctggccaaggcgtggcctggaccaaaatgcccgtctgc

SEQ ID NO: 70 - DNA, 2274 bp, synthetic construct
  source 1..2274: mol_type = other DNA
tgcggcagcccccctcccatcctgaacggcagaatcagctactacagcacccccatcgccgtgggcaccgtgatcagatacagctgcagcggcaccttcgccctgatcggcgaggctagcctgctgtgcatcaccaaggacaaggtggacggcacctgggacaagcccgcccccaagtgcgagtacttcaacgcctacagcagctgccccgagcccatcgtgcctggcggctacaagatcagaggcagcaccccctacagacacggcgacagcgtgaccttcgcctgcaagaccaacttcagcatgaacggcaacaagagcgtgtggtgccaagccaacaacatgtggggccccacaagactgcccacctgcgtgagcgtgttccccctggagtgccccgccctgcccatgatccacaacggccaccacacaagcgagaacgtgggcagcatcgcccccggcctgagcgtgacctacagctgcgagagcggctacctgctggtgggcgagaagatcatcaactgcctgagcagcggcaagtggagcgccgtgccccccacctgcgaggaggctagatgcaagagcctgggcagattccccaacggcaaggtgaaggagcctcctatcctgagagtgggcgtgaccgccaacttcttctgcgacgagggctacagactgcaaggcccccctagcagcagatgtgtgatcgctggccaaggcgtggcctggaccaaaatgcccgtctgcgggggggggggcagcgggggcgggggcagcgaggattgcaacgagctgccccctagacggaacacagagatcctgaccggcagctggagcgatcaaacatatcccgagggcacccaagccatctacaaatgcagacctggctacagaagcctgggcaatgtgatcatggtctgccggaaaggggagtgggtcgctctgaaccccctgcggaagtgtcagaagagaccttgcggccaccccggcgacacacccttcgggaccttcacactgaccggcggcaacgtgtttgagtacggcgtcaaggccgtgtacacctgtaacgaggggtatcagctgctgggcgagatcaactacagagagtgcgataccgacggctggaccaatgacatccccatctgcgaggtggtgaagtgtctgcccgtgaccgcccccgaaaacggcaagatcgtgagcagcgccatggagcccgaccgggagtaccattttgggcaagctgtgagattcgtctgcaatagcggctacaagatcgaaggcgacgaggagatgcactgtagcgacgacggcttctggtccaaagagaaacccaaatgcgtggagatctcctgcaaaagccccgatgtgatcaacggcagccccatctcccaaaaaattatctacaaggaaaacgaacggtttcagtacaaatgcaacatgggctacgaatactccgagcggggggatgccgtgtgcaccgagagcggctggcggcctctgcctagctgtgaagggggcggcgggagcggcgggggcggcagcgaggactgcaatgaactgcctcctagacggaacaccgaaatcctgaccgggagctggagcgaccaaacataccccgaggggacacaagccatctacaagtgcagacctgggtatagatccctcgggaacgtgatcatggtctgtcggaagggcgagtgggtcgctctgaaccctctcagaaagtgtcagaaacggccctgcgggcaccccggcgatacccccttcggcacattcaccctgaccggggggaacgtgttcgagtacggcgtgaaggccgtctacacctgcaacgagggctaccaactcctgggcgaaatcaattacagagaatgcgacacagatggctggaccaacgacatccctatctgcgaggtcgtgaaatgtctccccgtgacagcccctgagaacggcaagattgtcagcagcgctatggaacctgatagagagtaccatttcggccaagccgtcagatttgtgtgcaattccggctacaaaattgagggggacgaagagatgcactgctccgacgatggcttctggagcaaggaaaaacccaagtgcgtggagattagctgcaagagccccgacgtgatcaacgggagccccatctcccaaaaaatcatctacaaggagaacgagagatttcagtataagtgcaacatgggctatgagtacagcgagcggggggacgccgtgtgtaccgaatccgggtggagacccctgcctagctgc

SEQ ID NO: 71 - DNA, 2355 bp, synthetic construct
  source 1..2355: mol_type = other DNA
atgcccatgggcagcctgcagcccctggccaccctgtacctgctgggcatgctggtggctagctgcctgggcatcagctgcggcagcccccctcccatcctgaacggcagaatcagctactacagcacccccatcgccgtgggcaccgtgatcagatacagctgcagcggcaccttcgccctgatcggcgaggctagcctgctgtgcatcaccaaggacaaggtggacggcacctgggacaagcccgcccccaagtgcgagtacttcaacgcctacagcagctgccccgagcccatcgtgcctggcggctacaagatcagaggcagcaccccctacagacacggcgacagcgtgaccttcgcctgcaagaccaacttcagcatgaacggcaacaagagcgtgtggtgccaagccaacaacatgtggggccccacaagactgcccacctgcgtgagcgtgttccccctggagtgccccgccctgcccatgatccacaacggccaccacacaagcgagaacgtgggcagcatcgcccccggcctgagcgtgacctacagctgcgagagcggctacctgctggtgggcgagaagatcatcaactgcctgagcagcggcaagtggagcgccgtgccccccacctgcgaggaggctagatgcaagagcctgggcagattccccaacggcaaggtgaaggagcctcctatcctgagagtgggcgtgaccgccaacttcttctgcgacgagggctacagactgcaaggcccccctagcagcagatgtgtgatcgctggccaaggcgtggcctggaccaaaatgcccgtctgcgggggggggggcagcgggggcgggggcagcgaggattgcaacgagctgccccctagacggaacacagagatcctgaccggcagctggagcgatcaaacatatcccgagggcacccaagccatctacaaatgcagacctggctacagaagcctgggcaatgtgatcatggtctgccggaaaggggagtgggtcgctctgaaccccctgcggaagtgtcagaagagaccttgcggccaccccggcgacacacccttcgggaccttcacactgaccggcggcaacgtgtttgagtacggcgtcaaggccgtgtacacctgtaacgaggggtatcagctgctgggcgagatcaactacagagagtgcgataccgacggctggaccaatgacatccccatctgcgaggtggtgaagtgtctgcccgtgaccgcccccgaaaacggcaagatcgtgagcagcgccatggagcccgaccgggagtaccattttgggcaagctgtgagattcgtctgcaatagcggctacaagatcgaaggcgacgaggagatgcactgtagcgacgacggcttctggtccaaagagaaacccaaatgcgtggagatctcctgcaaaagccccgatgtgatcaacggcagccccatctcccaaaaaattatctacaaggaaaacgaacggtttcagtacaaatgcaacatgggctacgaatactccgagcggggggatgccgtgtgcaccgagagcggctggcggcctctgcctagctgtgaagggggcggcgggagcggcgggggcggcagcgaggactgcaatgaactgcctcctagacggaacaccgaaatcctgaccgggagctggagcgaccaaacataccccgaggggacacaagccatctacaagtgcagacctgggtatagatccctcgggaacgtgatcatggtctgtcggaagggcgagtgggtcgctctgaaccctctcagaaagtgtcagaaacggccctgcgggcaccccggcgatacccccttcggcacattcaccctgaccggggggaacgtgttcgagtacggcgtgaaggccgtctacacctgcaacgagggctaccaactcctgggcgaaatcaattacagagaatgcgacacagatggctggaccaacgacatccctatctgcgaggtcgtgaaatgtctccccgtgacagcccctgagaacggcaagattgtcagcagcgctatggaacctgatagagagtaccatttcggccaagccgtcagatttgtgtgcaattccggctacaaaattgagggggacgaagagatgcactgctccgacgatggcttctggagcaaggaaaaacccaagtgcgtggagattagctgcaagagccccgacgtgatcaacgggagccccatctcccaaaaaatcatctacaaggagaacgagagatttcagtataagtgcaacatgggctatgagtacagcgagcggggggacgccgtgtgtaccgaatccgggtggagacccctgcctagctgcgag

SEQ ID NO: 72 - DNA, 1893 bp, synthetic construct
  source 1..1893: mol_type = other DNA
tgtggcagccctcctcctattctgaatggcaggatcagctactacagcacccctattgccgtgggcaccgtgatcagatacagctgctctggcacattcgccctgatcggcgaagccagcctgctgtgcatcaccaaggataaggtggacggcacctgggacaagcccgctcctaagtgcgaatatttcaacgcctacagcagctgccctgagcctattgtgcctggcggctacaagatcagaggcagcaccccatacagacacggcgacagcgtgacctttgcctgcaagaccaacttcagcatgaacggcaacaagagcgtgtggtgccaggccaacaatatgtggggccctaccagactgcccacctgtgtgtctgtgttccctctggaatgccccgctctgcccatgatccacaatggccaccacaccagcgagaacgtgggatctattgcccctggcctgtccgtgacctacagctgtgaaagcggctatctgctcgtgggcgagaagatcatcaactgcctgagcagcggcaagtggagcgctgttcctcctacatgcgaagaggccagatgcaagagcctgggcagattccccaacggcaaagtgaaagagcctcctatcctgagagtgggcgtgaccgccaacttcttctgcgacgagggctacagactgcagggccctcctagcagcagatgtgtgattgctggacagggcgtcgcctggaccaagatgcctgtttgtggcggaggtgggtcgggtggcggcggatctgaggactgcaacgaactgcctcctagaagaaacaccgaaatcctcacaggctcctggtcagatcagacctaccctgagggtacacaggccatctataaatgccgcccgggttaccgctccttgggcaatgttattatggtctgccggaaaggggaatgggtggccttgaaccccctcagaaagtgccaaaaaagaccctgcggacatccaggagacacacctttcgggacatttaccttgaccggtggtaacgtgttcgagtacggagtgaaggcagtctatacttgcaatgagggctaccagctcctgggggaaataaattatcgcgaatgtgatacagacggctggacgaacgacattcctatctgtgaggtggtcaaatgtctgcccgtcactgctcctgaaaacggcaagatagtgagttctgcaatggagccggatagggagtatcattttggtcaggccgtgcgctttgtgtgcaatagtgggtataaaatcgagggggatgaagaaatgcactgtagcgacgatggattctggtctaaagagaaacctaagtgtgtggagattagttgcaagagtccagacgtgattaacggtagccccatttcccaaaagataatatacaaggaaaacgaaagattccagtataaatgcaacatgggctacgagtatagcgagcggggcgatgccgtgtgtactgaaagcggctggcgccccctgccttcctgcgagcgggatacaagctgcgtgaaccctccaacagtccaaaatgcctatatagtctctaggcagatgagtaaatacccaagtggagagagagtgagataccagtgccggtctccttacgagatgttcggcgacgaggaagtgatgtgcctgaacggcaattggacagagccaccacaatgtaaggatagtacaggcaaatgtgtgatcagtcgggagatcatggagaactacaacattgccctgaggtggactgctaagcagaagctctatagccgaacaggcgagtcagtggagtttgtgtgtaaacggggatacaggctgtccagtaggagccacaccctgcgcactacttgctgggatgggaagctggaatatccaacttgc

SEQ ID NO: 73 - DNA, 1980 bp, synthetic construct
  source 1..1980: mol_type = other DNA
atgccaatggggtccctacaacccctggcaacactatatctgctaggtatgctcgtggcctcctgtttaggaatcagctgtggcagccctcctcctattctgaatggcaggatcagctactacagcacccctattgccgtgggcaccgtgatcagatacagctgctctggcacattcgccctgatcggcgaagccagcctgctgtgcatcaccaaggataaggtggacggcacctgggacaagcccgctcctaagtgcgaatatttcaacgcctacagcagctgccctgagcctattgtgcctggcggctacaagatcagaggcagcaccccatacagacacggcgacagcgtgacctttgcctgcaagaccaacttcagcatgaacggcaacaagagcgtgtggtgccaggccaacaatatgtggggccctaccagactgcccacctgtgtgtctgtgttccctctggaatgccccgctctgcccatgatccacaatggccaccacaccagcgagaacgtgggatctattgcccctggcctgtccgtgacctacagctgtgaaagcggctatctgctcgtgggcgagaagatcatcaactgcctgagcagcggcaagtggagcgctgttcctcctacatgcgaagaggccagatgcaagagcctgggcagattccccaacggcaaagtgaaagagcctcctatcctgagagtgggcgtgaccgccaacttcttctgcgacgagggctacagactgcagggccctcctagcagcagatgtgtgattgctggacagggcgtcgcctggaccaagatgcctgtttgtggcggaggtgggtcgggtggcggcggatctgaggactgcaacgaactgcctcctagaagaaacaccgaaatcctcacaggctcctggtcagatcagacctaccctgagggtacacaggccatctataaatgccgcccgggttaccgctccttgggcaatgttattatggtctgccggaaaggggaatgggtggccttgaaccccctcagaaagtgccaaaaaagaccctgcggacatccaggagacacacctttcgggacatttaccttgaccggtggtaacgtgttcgagtacggagtgaaggcagtctatacttgcaatgagggctaccagctcctgggggaaataaattatcgcgaatgtgatacagacggctggacgaacgacattcctatctgtgaggtggtcaaatgtctgcccgtcactgctcctgaaaacggcaagatagtgagttctgcaatggagccggatagggagtatcattttggtcaggccgtgcgctttgtgtgcaatagtgggtataaaatcgagggggatgaagaaatgcactgtagcgacgatggattctggtctaaagagaaacctaagtgtgtggagattagttgcaagagtccagacgtgattaacggtagccccatttcccaaaagataatatacaaggaaaacgaaagattccagtataaatgcaacatgggctacgagtatagcgagcggggcgatgccgtgtgtactgaaagcggctggcgccccctgccttcctgcgagcgggatacaagctgcgtgaaccctccaacagtccaaaatgcctatatagtctctaggcagatgagtaaatacccaagtggagagagagtgagataccagtgccggtctccttacgagatgttcggcgacgaggaagtgatgtgcctgaacggcaattggacagagccaccacaatgtaaggatagtacaggcaaatgtgtgatcagtcgggagatcatggagaactacaacattgccctgaggtggactgctaagcagaagctctatagccgaacaggcgagtcagtggagtttgtgtgtaaacggggatacaggctgtccagtaggagccacaccctgcgcactacttgctgggatgggaagctggaatatccaacttgcgccaagagg

SEQ ID NO: 74 - DNA, 2478 bp, synthetic construct
  source 1..2478: mol_type = other DNA
tgcggcagcccccctcccatcctgaacggcagaatcagctactacagcacccccatcgccgtgggcaccgtgatcagatacagctgcagcggcaccttcgccctgatcggcgaggctagcctgctgtgcatcaccaaggacaaggtggacggcacctgggacaagcccgcccccaagtgcgagtacttcaacgcctacagcagctgccccgagcccatcgtgcctggcggctacaagatcagaggcagcaccccctacagacacggcgacagcgtgaccttcgcctgcaagaccaacttcagcatgaacggcaacaagagcgtgtggtgccaagccaacaacatgtggggccccacaagactgcccacctgcgtgagcgtgttccccctggagtgccccgccctgcccatgatccacaacggccaccacacaagcgagaacgtgggcagcatcgcccccggcctgagcgtgacctacagctgcgagagcggctacctgctggtgggcgagaagatcatcaactgcctgagcagcggcaagtggagcgccgtgccccccacctgcgaggaggctagatgcaagagcctgggcagattccccaacggcaaggtgaaggagcctcctatcctgagagtgggcgtgaccgccaacttcttctgcgacgagggctacagactgcaaggcccccctagcagcagatgtgtgatcgctggccaaggcgtggcctggaccaaaatgcccgtctgcgggggggggggcagcgggggcgggggcagcgaggattgcaacgagctgccccctagacggaacacagagatcctgaccggcagctggagcgatcaaacatatcccgagggcacccaagccatctacaaatgcagacctggctacagaagcctgggcaatgtgatcatggtctgccggaaaggggagtgggtcgctctgaaccccctgcggaagtgtcagaagagaccttgcggccaccccggcgacacacccttcgggaccttcacactgaccggcggcaacgtgtttgagtacggcgtcaaggccgtgtacacctgtaacgaggggtatcagctgctgggcgagatcaactacagagagtgcgataccgacggctggaccaatgacatccccatctgcgaggtggtgaagtgtctgcccgtgaccgcccccgaaaacggcaagatcgtgagcagcgccatggagcccgaccgggagtaccattttgggcaagctgtgagattcgtctgcaatagcggctacaagatcgaaggcgacgaggagatgcactgtagcgacgacggcttctggtccaaagagaaacccaaatgcgtggagatctcctgcaaaagccccgatgtgatcaacggcagccccatctcccaaaaaattatctacaaggaaaacgaacggtttcagtacaaatgcaacatgggctacgaatactccgagcggggggatgccgtgtgcaccgagagcggctggcggcctctgcctagctgtgaagggggcggcgggagcggcgggggcggcagcgaggactgcaatgaactgcctcctagacggaacaccgaaatcctgaccgggagctggagcgaccaaacataccccgaggggacacaagccatctacaagtgcagacctgggtatagatccctcgggaacgtgatcatggtctgtcggaagggcgagtgggtcgctctgaaccctctcagaaagtgtcagaaacggccctgcgggcaccccggcgatacccccttcggcacattcaccctgaccggggggaacgtgttcgagtacggcgtgaaggccgtctacacctgcaacgagggctaccaactcctgggcgaaatcaattacagagaatgcgacacagatggctggaccaacgacatccctatctgcgaggtcgtgaaatgtctccccgtgacagcccctgagaacggcaagattgtcagcagcgctatggaacctgatagagagtaccatttcggccaagccgtcagatttgtgtgcaattccggctacaaaattgagggggacgaagagatgcactgctccgacgatggcttctggagcaaggaaaaacccaagtgcgtggagattagctgcaagagccccgacgtgatcaacgggagccccatctcccaaaaaatcatctacaaggagaacgagagatttcagtataagtgcaacatgggctatgagtacagcgagcggggggacgccgtgtgtaccgaatccgggtggagacccctgcctagctgcgagggcgggggcgggagcggcgggggcggctccctgagaaagtgttacttcccctacctggagaacggctacaatcagaaccacggcagaaagttcgtgcaaggcaagagcatcgacgtggcctgccaccccggctacgccctgcccaaggctcagaccaccgtgacctgcatggagaatggctggagccccacccctagatgc

SEQ ID NO: 75 - DNA, 2571 bp, synthetic construct
  source 1..2571: mol_type = other DNA
atgcccatgggcagcctgcagcccctggccaccctgtacctgctgggcatgctggtggctagctgcctgggcatcagctgcggcagcccccctcccatcctgaacggcagaatcagctactacagcacccccatcgccgtgggcaccgtgatcagatacagctgcagcggcaccttcgccctgatcggcgaggctagcctgctgtgcatcaccaaggacaaggtggacggcacctgggacaagcccgcccccaagtgcgagtacttcaacgcctacagcagctgccccgagcccatcgtgcctggcggctacaagatcagaggcagcaccccctacagacacggcgacagcgtgaccttcgcctgcaagaccaacttcagcatgaacggcaacaagagcgtgtggtgccaagccaacaacatgtggggccccacaagactgcccacctgcgtgagcgtgttccccctggagtgccccgccctgcccatgatccacaacggccaccacacaagcgagaacgtgggcagcatcgcccccggcctgagcgtgacctacagctgcgagagcggctacctgctggtgggcgagaagatcatcaactgcctgagcagcggcaagtggagcgccgtgccccccacctgcgaggaggctagatgcaagagcctgggcagattccccaacggcaaggtgaaggagcctcctatcctgagagtgggcgtgaccgccaacttcttctgcgacgagggctacagactgcaaggcccccctagcagcagatgtgtgatcgctggccaaggcgtggcctggaccaaaatgcccgtctgcgggggggggggcagcgggggcgggggcagcgaggattgcaacgagctgccccctagacggaacacagagatcctgaccggcagctggagcgatcaaacatatcccgagggcacccaagccatctacaaatgcagacctggctacagaagcctgggcaatgtgatcatggtctgccggaaaggggagtgggtcgctctgaaccccctgcggaagtgtcagaagagaccttgcggccaccccggcgacacacccttcgggaccttcacactgaccggcggcaacgtgtttgagtacggcgtcaaggccgtgtacacctgtaacgaggggtatcagctgctgggcgagatcaactacagagagtgcgataccgacggctggaccaatgacatccccatctgcgaggtggtgaagtgtctgcccgtgaccgcccccgaaaacggcaagatcgtgagcagcgccatggagcccgaccgggagtaccattttgggcaagctgtgagattcgtctgcaatagcggctacaagatcgaaggcgacgaggagatgcactgtagcgacgacggcttctggtccaaagagaaacccaaatgcgtggagatctcctgcaaaagccccgatgtgatcaacggcagccccatctcccaaaaaattatctacaaggaaaacgaacggtttcagtacaaatgcaacatgggctacgaatactccgagcggggggatgccgtgtgcaccgagagcggctggcggcctctgcctagctgtgaagggggcggcgggagcggcgggggcggcagcgaggactgcaatgaactgcctcctagacggaacaccgaaatcctgaccgggagctggagcgaccaaacataccccgaggggacacaagccatctacaagtgcagacctgggtatagatccctcgggaacgtgatcatggtctgtcggaagggcgagtgggtcgctctgaaccctctcagaaagtgtcagaaacggccctgcgggcaccccggcgatacccccttcggcacattcaccctgaccggggggaacgtgttcgagtacggcgtgaaggccgtctacacctgcaacgagggctaccaactcctgggcgaaatcaattacagagaatgcgacacagatggctggaccaacgacatccctatctgcgaggtcgtgaaatgtctccccgtgacagcccctgagaacggcaagattgtcagcagcgctatggaacctgatagagagtaccatttcggccaagccgtcagatttgtgtgcaattccggctacaaaattgagggggacgaagagatgcactgctccgacgatggcttctggagcaaggaaaaacccaagtgcgtggagattagctgcaagagccccgacgtgatcaacgggagccccatctcccaaaaaatcatctacaaggagaacgagagatttcagtataagtgcaacatgggctatgagtacagcgagcggggggacgccgtgtgtaccgaatccgggtggagacccctgcctagctgcgagggcgggggcgggagcggcgggggcggctccctgagaaagtgttacttcccctacctggagaacggctacaatcagaaccacggcagaaagttcgtgcaaggcaagagcatcgacgtggcctgccaccccggctacgccctgcccaaggctcagaccaccgtgacctgcatggagaatggctggagccccacccctagatgcatcagagtgaagacc

SEQ ID NO: 76 - DNA, 747 bp, synthetic construct
  source 1..747: mol_type = other DNA
tgcggcagcccccctcccatcctcaacggcagaatcagctactacagcacccccatcgccgtgggcaccgtgatcagatacagctgcagcggcaccttcagactgatcggcgagaagagcctgctgtgcatcaccaaggacaaggtggacggcacctgggacaagcccgcccccaagtgcgagtacttcaacaagtacagcagctgccccgagcccatcgtgcccggcggctataagatcagaggcagcaccccctacagacacggcgacagcgtgaccttcgcctgcaagaccaacttcagcatgaacggcaacaagagcgtgtggtgccaagccaacaacatgtggggccccacaagactgcccacctgcgtgagcgtgttccccctggagtgccccgccctgcccatgatccacaacggccaccacacaagcgagaacgtgggcagcatcgcccccggcctgagcgtgacctacagctgcgagagcggctacctgctggtgggcgagaagatcatcaactgcctgagcagcggcaagtggagcgccgtgccccccacctgcgaggaggctagatgcaagagcctgggcagattccccaacggcaaggtgaaggagccccccatcctgagagtgggcgtgaccgccaacttcttctgcgacgagggctacagactgcaaggcccccctagcagcagatgcgtgatcgccggccaaggcgtggcttggacaaaaatgcctgtgtgt

SEQ ID NO: 77 - DNA, 900 bp, synthetic construct
  source 1..900: mol_type = other DNA
tgcaatgagctccccccccggagaaacaccgagatcctgaccggcagctggagcgatcagacctatcccgagggcacccaagccatttataagtgcagacccggctacagaagcctggggaatgtgatcatggtctgcagaaagggcgagtgggtggccctgaatcccctccggaagtgccaaaagcggccctgtgggcaccccggcgacacacccttcggcacctttaccctgaccggcggcaatgtcttcgagtatggcgtcaaggccgtgtatacctgcaacgaaggctatcagctgctgggcgagatcaactatcgggagtgtgacaccgacggctggacaaacgacatccccatctgcgaggtggtgaagtgcctgcccgtgaccgcccccgaaaacggcaaaatcgtcagcagcgctatggaacccgaccgggaataccacttcggccaagctgtcagattcgtgtgtaatagcgggtataagattgagggcgatgaggaaatgcactgcagcgacgacggcttctggagcaaggagaagcccaaatgcgtggagatcagctgtaaaagccccgacgtgatcaacggcagccccatcagccaaaaaatcatttacaaggagaacgaaagatttcagtacaagtgtaatatgggctacgagtatagcgagcggggcgacgctgtgtgcaccgagagcggctggagacctctcccttcctgcgaggagaagagctgcgacaacccctacatccccaacggcgactactcccccctgagaatcaaacatagaaccggggacgagatcacctatcagtgcagaaatggcttctaccctgccacaagagggaacaccgccaagtgcacatccaccgggtggattcccgctcctagatgt

SEQ ID NO: 78 - DNA, 900 bp, synthetic construct
  source 1..900: mol_type = other DNA
tgcaacgagctgccccctcggagaaacacagagatcctgaccgggagctggagcgatcagacctaccccgaggggacacaagccatctacaagtgcagacctgggtatagaagcctgggcaacgtgattatggtgtgcagaaagggggaatgggtggccctgaatcccctgagaaagtgtcagaagagaccctgcggccaccctggcgatacaccctttggcaccttcaccctgaccgggggcaacgtgttcgagtacggcgtgaaggccgtgtacacatgcaacgagggctatcaactgctgggggagatcaattacagagagtgcgataccgatgggtggaccaacgacattcctatctgcgaagtcgtgaagtgcctccctgtcaccgcccccgagaacggcaagatcgtgagcagcgctatggagcctgatagagagtaccactttgggcaagccgtgagattcgtctgcaacagcgggtacaagatcgagggcgacgaggagatgcactgttccgatgacgggttctggagcaaagagaagcccaagtgtgtggagatcagctgcaaaagccccgatgtgatcaatggcagccccattagccaaaagattatctataaggaaaacgagagattccaatacaagtgcaacatggggtacgagtactccgaaagaggcgacgccgtctgcaccgaatccggctggagacctctccctagctgtgaggagaagagctgtgataacccctatattcccaacggcgattattcccctctgagaatcaagcaccggaccggcgacgagattacctatcagtgtagaaacggcttctaccccgctacaagaggcaataccgctaagtgcacctccaccggctggattcccgcccctagatgc

SEQ ID NO: 79 - protein, 876 aa, synthetic construct
CGSPPPILNGRISYYSTPIAVGTVIRYSCSGTFRLIGEKSLLCITKDKVDGTWDKPAPKCEYFNKYSSCPEPIVPGGYKIRGSTPYRHGDSVTFACKTNFSMNGNKSVWCQANNMWGPTRLPTCVSVFPLECPALPMIHNGHHTSENVGSIAPGLSVTYSCESGYLLVGEKIINCLSSGKWSAVPPTCEEARCKSLGRFPNGKVKEPPILRVGVTANFFCDEGYRLQGPPSSRCVIAGQGVAWTKMPVCGGGGSGGGGSEDCNELPPRRNTEILTGSWSDQTYPEGTQAIYKCRPGYRSLGNVIMVCRKGEWVALNPLRKCQKRPCGHPGDTPFGTFTLTGGNVFEYGVKAVYTCNEGYQLLGEINYRECDTDGWTNDIPICEVVKCLPVTAPENGKIVSSAMEPDREYHFGQAVRFVCNSGYKIEGDEEMHCSDDGFWSKEKPKCVEISCKSPDVINGSPISQKIIYKENERFQYKCNMGYEYSERGDAVCTESGWRPLPSCEEKSCDNPYIPNGDYSPLRIKHRTGDEITYQCRNGFYPATRGNTAKCTSTGWIPAPRCTLKGGGGSGGGGSEDCNELPPRRNTEILTGSWSDQTYPEGTQAIYKCRPGYRSLGNVIMVCRKGEWVALNPLRKCQKRPCGHPGDTPFGTFTLTGGNVFEYGVKAVYTCNEGYQLLGEINYRECDTDGWTNDIPICEVVKCLPVTAPENGKIVSSAMEPDREYHFGQAVRFVCNSGYKIEGDEEMHCSDDGFWSKEKPKCVEISCKSPDVINGSPISQKIIYKENERFQYKCNMGYEYSERGDAVCTESGWRPLPSCEEKSCDNPYIPNGDYSPLRIKHRTGDEITYQCRNGFYPATRGNTAKCTSTGWIPAPRC

SEQ ID NO: 80 - DNA, 2628 bp, synthetic construct
  source 1..2628: mol_type = other DNA
tgcggcagcccccctcccatcctcaacggcagaatcagctactacagcacccccatcgccgtgggcaccgtgatcagatacagctgcagcggcaccttcagactgatcggcgagaagagcctgctgtgcatcaccaaggacaaggtggacggcacctgggacaagcccgcccccaagtgcgagtacttcaacaagtacagcagctgccccgagcccatcgtgcccggcggctataagatcagaggcagcaccccctacagacacggcgacagcgtgaccttcgcctgcaagaccaacttcagcatgaacggcaacaagagcgtgtggtgccaagccaacaacatgtggggccccacaagactgcccacctgcgtgagcgtgttccccctggagtgccccgccctgcccatgatccacaacggccaccacacaagcgagaacgtgggcagcatcgcccccggcctgagcgtgacctacagctgcgagagcggctacctgctggtgggcgagaagatcatcaactgcctgagcagcggcaagtggagcgccgtgccccccacctgcgaggaggctagatgcaagagcctgggcagattccccaacggcaaggtgaaggagccccccatcctgagagtgggcgtgaccgccaacttcttctgcgacgagggctacagactgcaaggcccccctagcagcagatgcgtgatcgccggccaaggcgtggcttggacaaaaatgcctgtgtgtggcgggggcgggagcggcgggggcggcagcgaagactgcaatgagctccccccccggagaaacaccgagatcctgaccggcagctggagcgatcagacctatcccgagggcacccaagccatttataagtgcagacccggctacagaagcctggggaatgtgatcatggtctgcagaaagggcgagtgggtggccctgaatcccctccggaagtgccaaaagcggccctgtgggcaccccggcgacacacccttcggcacctttaccctgaccggcggcaatgtcttcgagtatggcgtcaaggccgtgtatacctgcaacgaaggctatcagctgctgggcgagatcaactatcgggagtgtgacaccgacggctggacaaacgacatccccatctgcgaggtggtgaagtgcctgcccgtgaccgcccccgaaaacggcaaaatcgtcagcagcgctatggaacccgaccgggaataccacttcggccaagctgtcagattcgtgtgtaatagcgggtataagattgagggcgatgaggaaatgcactgcagcgacgacggcttctggagcaaggagaagcccaaatgcgtggagatcagctgtaaaagccccgacgtgatcaacggcagccccatcagccaaaaaatcatttacaaggagaacgaaagatttcagtacaagtgtaatatgggctacgagtatagcgagcggggcgacgctgtgtgcaccgagagcggctggagacctctcccttcctgcgaggagaagagctgcgacaacccctacatccccaacggcgactactcccccctgagaatcaaacatagaaccggggacgagatcacctatcagtgcagaaatggcttctaccctgccacaagagggaacaccgccaagtgcacatccaccgggtggattcccgctcctagatgtacactcaagggcgggggcggcagcggcgggggcggcagcgaggactgcaacgagctgccccctcggagaaacacagagatcctgaccgggagctggagcgatcagacctaccccgaggggacacaagccatctacaagtgcagacctgggtatagaagcctgggcaacgtgattatggtgtgcagaaagggggaatgggtggccctgaatcccctgagaaagtgtcagaagagaccctgcggccaccctggcgatacaccctttggcaccttcaccctgaccgggggcaacgtgttcgagtacggcgtgaaggccgtgtacacatgcaacgagggctatcaactgctgggggagatcaattacagagagtgcgataccgatgggtggaccaacgacattcctatctgcgaagtcgtgaagtgcctccctgtcaccgcccccgagaacggcaagatcgtgagcagcgctatggagcctgatagagagtaccactttgggcaagccgtgagattcgtctgcaacagcgggtacaagatcgagggcgacgaggagatgcactgttccgatgacgggttctggagcaaagagaagcccaagtgtgtggagatcagctgcaaaagccccgatgtgatcaatggcagccccattagccaaaagattatctataaggaaaacgagagattccaatacaagtgcaacatggggtacgagtactccgaaagaggcgacgccgtctgcaccgaatccggctggagacctctccctagctgtgaggagaagagctgtgataacccctatattcccaacggcgattattcccctctgagaatcaagcaccggaccggcgacgagattacctatcagtgtagaaacggcttctaccccgctacaagaggcaataccgctaagtgcacctccaccggctggattcccgcccctagatgc

SEQ ID NO: 81 - protein, 905 aa, synthetic construct
MPMGSLQPLATLYLLGMLVASCLGISCGSPPPILNGRISYYSTPIAVGTVIRYSCSGTFRLIGEKSLLCITKDKVDGTWDKPAPKCEYFNKYSSCPEPIVPGGYKIRGSTPYRHGDSVTFACKTNFSMNGNKSVWCQANNMWGPTRLPTCVSVFPLECPALPMIHNGHHTSENVGSIAPGLSVTYSCESGYLLVGEKIINCLSSGKWSAVPPTCEEARCKSLGRFPNGKVKEPPILRVGVTANFFCDEGYRLQGPPSSRCVIAGQGVAWTKMPVCGGGGSGGGGSEDCNELPPRRNTEILTGSWSDQTYPEGTQAIYKCRPGYRSLGNVIMVCRKGEWVALNPLRKCQKRPCGHPGDTPFGTFTLTGGNVFEYGVKAVYTCNEGYQLLGEINYRECDTDGWTNDIPICEVVKCLPVTAPENGKIVSSAMEPDREYHFGQAVRFVCNSGYKIEGDEEMHCSDDGFWSKEKPKCVEISCKSPDVINGSPISQKIIYKENERFQYKCNMGYEYSERGDAVCTESGWRPLPSCEEKSCDNPYIPNGDYSPLRIKHRTGDEITYQCRNGFYPATRGNTAKCTSTGWIPAPRCTLKGGGGSGGGGSEDCNELPPRRNTEILTGSWSDQTYPEGTQAIYKCRPGYRSLGNVIMVCRKGEWVALNPLRKCQKRPCGHPGDTPFGTFTLTGGNVFEYGVKAVYTCNEGYQLLGEINYRECDTDGWTNDIPICEVVKCLPVTAPENGKIVSSAMEPDREYHFGQAVRFVCNSGYKIEGDEEMHCSDDGFWSKEKPKCVEISCKSPDVINGSPISQKIIYKENERFQYKCNMGYEYSERGDAVCTESGWRPLPSCEEKSCDNPYIPNGDYSPLRIKHRTGDEITYQCRNGFYPATRGNTAKCTSTGWIPAPRCTLK

SEQ ID NO: 82 - DNA, 2715 bp, synthetic construct
  source 1..2715: mol_type = other DNA
atgcccatgggcagcctgcagcccctggccaccctgtacctgctgggcatgctggtggctagctgcctgggcatcagctgcggcagcccccctcccatcctcaacggcagaatcagctactacagcacccccatcgccgtgggcaccgtgatcagatacagctgcagcggcaccttcagactgatcggcgagaagagcctgctgtgcatcaccaaggacaaggtggacggcacctgggacaagcccgcccccaagtgcgagtacttcaacaagtacagcagctgccccgagcccatcgtgcccggcggctataagatcagaggcagcaccccctacagacacggcgacagcgtgaccttcgcctgcaagaccaacttcagcatgaacggcaacaagagcgtgtggtgccaagccaacaacatgtggggccccacaagactgcccacctgcgtgagcgtgttccccctggagtgccccgccctgcccatgatccacaacggccaccacacaagcgagaacgtgggcagcatcgcccccggcctgagcgtgacctacagctgcgagagcggctacctgctggtgggcgagaagatcatcaactgcctgagcagcggcaagtggagcgccgtgccccccacctgcgaggaggctagatgcaagagcctgggcagattccccaacggcaaggtgaaggagccccccatcctgagagtgggcgtgaccgccaacttcttctgcgacgagggctacagactgcaaggcccccctagcagcagatgcgtgatcgccggccaaggcgtggcttggacaaaaatgcctgtgtgtggcgggggcgggagcggcgggggcggcagcgaagactgcaatgagctccccccccggagaaacaccgagatcctgaccggcagctggagcgatcagacctatcccgagggcacccaagccatttataagtgcagacccggctacagaagcctggggaatgtgatcatggtctgcagaaagggcgagtgggtggccctgaatcccctccggaagtgccaaaagcggccctgtgggcaccccggcgacacacccttcggcacctttaccctgaccggcggcaatgtcttcgagtatggcgtcaaggccgtgtatacctgcaacgaaggctatcagctgctgggcgagatcaactatcgggagtgtgacaccgacggctggacaaacgacatccccatctgcgaggtggtgaagtgcctgcccgtgaccgcccccgaaaacggcaaaatcgtcagcagcgctatggaacccgaccgggaataccacttcggccaagctgtcagattcgtgtgtaatagcgggtataagattgagggcgatgaggaaatgcactgcagcgacgacggcttctggagcaaggagaagcccaaatgcgtggagatcagctgtaaaagccccgacgtgatcaacggcagccccatcagccaaaaaatcatttacaaggagaacgaaagatttcagtacaagtgtaatatgggctacgagtatagcgagcggggcgacgctgtgtgcaccgagagcggctggagacctctcccttcctgcgaggagaagagctgcgacaacccctacatccccaacggcgactactcccccctgagaatcaaacatagaaccggggacgagatcacctatcagtgcagaaatggcttctaccctgccacaagagggaacaccgccaagtgcacatccaccgggtggattcccgctcctagatgtacactcaagggcgggggcggcagcggcgggggcggcagcgaggactgcaacgagctgccccctcggagaaacacagagatcctgaccgggagctggagcgatcagacctaccccgaggggacacaagccatctacaagtgcagacctgggtatagaagcctgggcaacgtgattatggtgtgcagaaagggggaatgggtggccctgaatcccctgagaaagtgtcagaagagaccctgcggccaccctggcgatacaccctttggcaccttcaccctgaccgggggcaacgtgttcgagtacggcgtgaaggccgtgtacacatgcaacgagggctatcaactgctgggggagatcaattacagagagtgcgataccgatgggtggaccaacgacattcctatctgcgaagtcgtgaagtgcctccctgtcaccgcccccgagaacggcaagatcgtgagcagcgctatggagcctgatagagagtaccactttgggcaagccgtgagattcgtctgcaacagcgggtacaagatcgagggcgacgaggagatgcactgttccgatgacgggttctggagcaaagagaagcccaagtgtgtggagatcagctgcaaaagccccgatgtgatcaatggcagccccattagccaaaagattatctataaggaaaacgagagattccaatacaagtgcaacatggggtacgagtactccgaaagaggcgacgccgtctgcaccgaatccggctggagacctctccctagctgtgaggagaagagctgtgataacccctatattcccaacggcgattattcccctctgagaatcaagcaccggaccggcgacgagattacctatcagtgtagaaacggcttctaccccgctacaagaggcaataccgctaagtgcacctccaccggctggattcccgcccctagatgcaccctcaag